European Patent Specification EP 3 582 808 B1, published February 7, 2024. Title: ENGINEERED BACTERIAL STRAIN THAT REDUCES ANTIBIOTIC-RESISTANT ENTEROCOCCUS COLONIZATION IN THE GI TRACT. Applicant: MEDICAL COLLEGE OF WISCONSIN Salzman, Nita Kristich, Christopher Kommineni, Sushma. The sequence listing filed with the application follows.

SEQUENCE LISTING (10 sequences)

SEQ ID NO: 1 - DNA, 2817 bp, Artificial Sequence
  synthetic
ttccagagaatcggatggtattaattttaaagaacaatcagtattctgaaaaacaaataaatgttctcgatcagttacaaaagttagattttaagattgaggaattagaaagtaccttacagatagaagatgagaggttcaatctggaagaatatcaagaagccatgattgatgaaaattatctttatgatatagatatcgtagaagaaaacaaagaagtagttcaagcgtataaccaggatagaatgaaagataagtcaaatgaaaatgaacaatttgaaggaattagtcatgatattgattgctaagaagtatctagtgacttttttcttgattgaaactcaagatagatatgttattgcttgcatcaaaataaactacatgggtataatagcaatgaaatgcatttccggacagatctcgacccgtgctataattatactaattttataaggaggaaaaaatatgggcatttttagtatttttgtaatcagcacagttcattatcaaccaaacaaaaaataagtggttataatgaatcgttaataagcaaaattcatataaccaaattaaagagggttataatgaacgagaaaaatataaaacacagtcaaaactttattacttcaaaacataatatagataaaataatgacaaatataagattaaatgaacatgataatatctttgaaatcggctcaggaaaaggccattttacccttgaattagtaaagaggtgtaatttcgtaactgccattgaaatagaccataaattatgcaaaactacagaaaataaacttgttgatcacgataatttccaagttttaaacaaggatatattgcagtttaaatttcctaaaaaccaatcctataaaatatatggtaatataccttataacataagtacggatataatacgcaaaattgtttttgatagtatagctaatgagatttatttaatcgtggaatacgggtttgctaaaagattattaaatacaaaacgctcattggcattacttttaatggcagaagttgatatttctatattaagtatggttccaagagaatattttcatcctaaacctaaagtgaatagctcacttatcagattaagtagaaaaaaatcaagaatatcacacaaagataaacaaaagtataattatttcgttatgaaatgggttaacaaagaatacaagaaaatatttacaaaaaatcaatttaacaattccttaaaacatgcaggaattgacgatttaaacaatattagctttgaacaattcttatctcttttcaatagctataaattatttaataagtaatgttgtacatgcgattagatatcattaattttgagaaatatttgaaaatttccttctatatatcaatatttattttttttctgggagtgttagcagggattataataggtcctcatataaataaattggactattttggtcaggaagtttcattttatagtgttagtgttaataatttaaaggtctctttttatttcctcactataggaatggtaacaggggggatttatgcatttttatttatgggtataaatggttatataattggtaagttgattcaatatttatacattaacaatgaactaaatgttttgtataaaggtcttcttccacatttttttatagagcttttaggattggcaacatttagtatgataagtaccattccaatatttgttattttggttttttttaaaacgcctacacatgtagttcctattaaaaaaatcataaagttaagtgtgttttttactgtacttggaatagttttaataataattggaggatatatagaatctaatataagctatgtagatatacgatagaagttgagatagaaaactaatctcaaaggaagatatccgcctatttccaaacgttatacgaaagaatttaaacaaaccattgatcacgaatcaaaaatgctgaattaaagatatactcattaaaggaagagtgggcactattttaaatttatacaaccaaggtaaaaattttcgtgaattatctttataataatatgtcggttacttaaaatttttgaaattcacaataaacatataattaacagtgtgataatttatttgtctacaagtcaattgggataggcaactctagttgcataaaatatctctcacaaaaagtgtttcatgtattactgaatctgatccatataagttcttaagaaaggaagataagtttgtacaagtttactttgaaaaaatacatcggtattacttcactattttttttgttttcaaatattctaattgctgaagagtttatttttgtagaaaaaaacttgagttttttccctaaattagggataattgtgcttgttttttttatgagtgctcccgcttttgttgttgttactttaattttgacttgtttagttgcatttcttattagtttaattaacaaattttacagtttcaaaagagtatacttatcgactttatttgtaaatagtattcagttattcgtaaatttagctttatttagtgtatttttacattacaatttaaatttgcgattgctaagtataatgagttttatgattaatatttttttagtagttatctatcgcaatttattaattaaatttgcgaatgtaaacagtagggctgcgaatgtattatcaattttcgggattgctttatctgtaatttatttggtggtaggagtaaagtaatgaaaaaaataacaattaacaacttgagtttttattatgaatccaaagatattatggtgtttgacaggttatctttagaatttt

SEQ ID NO: 2 - DNA, 909 bp, Artificial Sequence
  synthetic - ermC gene insert
cggacagatctcgacccgtgctataattatactaattttataaggaggaaaaaatatgggcatttttagtatttttgtaatcagcacagttcattatcaaccaaacaaaaaataagtggttataatgaatcgttaataagcaaaattcatataaccaaattaaagagggttataatgaacgagaaaaatataaaacacagtcaaaactttattacttcaaaacataatatagataaaataatgacaaatataagattaaatgaacatgataatatctttgaaatcggctcaggaaaaggccattttacccttgaattagtaaagaggtgtaatttcgtaactgccattgaaatagaccataaattatgcaaaactacagaaaataaacttgttgatcacgataatttccaagttttaaacaaggatatattgcagtttaaatttcctaaaaaccaatcctataaaatatatggtaatataccttataacataagtacggatataatacgcaaaattgtttttgatagtatagctaatgagatttatttaatcgtggaatacgggtttgctaaaagattattaaatacaaaacgctcattggcattacttttaatggcagaagttgatatttctatattaagtatggttccaagagaatattttcatcctaaacctaaagtgaatagctcacttatcagattaagtagaaaaaaatcaagaatatcacacaaagataaacaaaagtataattatttcgttatgaaatgggttaacaaagaatacaagaaaatatttacaaaaaatcaatttaacaattccttaaaacatgcaggaattgacgatttaaacaatattagctttgaacaattcttatctcttttcaatagctataaattatttaataagtaa

SEQ ID NO: 3 - DNA, 1908 bp, Artificial Sequence
  synthetic - PD1 backbone
ttccagagaatcggatggtattaattttaaagaacaatcagtattctgaaaaacaaataaatgttctcgatcagttacaaaagttagattttaagattgaggaattagaaagtaccttacagatagaagatgagaggttcaatctggaagaatatcaagaagccatgattgatgaaaattatctttatgatatagatatcgtagaagaaaacaaagaagtagttcaagcgtataaccaggatagaatgaaagataagtcaaatgaaaatgaacaatttgaaggaattagtcatgatattgattgctaagaagtatctagtgacttttttcttgattgaaactcaagatagatatgttattgcttgcatcaaaataaactacatgggtataatagcaatgaaatgcatttctgttgtacatgcgattagatatcattaattttgagaaatatttgaaaatttccttctatatatcaatatttattttttttctgggagtgttagcagggattataataggtcctcatataaataaattggactattttggtcaggaagtttcattttatagtgttagtgttaataatttaaaggtctctttttatttcctcactataggaatggtaacaggggggatttatgcatttttatttatgggtataaatggttatataattggtaagttgattcaatatttatacattaacaatgaactaaatgttttgtataaaggtcttcttccacatttttttatagagcttttaggattggcaacatttagtatgataagtaccattccaatatttgttattttggttttttttaaaacgcctacacatgtagttcctattaaaaaaatcataaagttaagtgtgttttttactgtacttggaatagttttaataataattggaggatatatagaatctaatataagctatgtagatatacgatagaagttgagatagaaaactaatctcaaaggaagatatccgcctatttccaaacgttatacgaaagaatttaaacaaaccattgatcacgaatcaaaaatgctgaattaaagatatactcattaaaggaagagtgggcactattttaaatttatacaaccaaggtaaaaattttcgtgaattatctttataataatatgtcggttacttaaaatttttgaaattcacaataaacatataattaacagtgtgataatttatttgtctacaagtcaattgggataggcaactctagttgcataaaatatctctcacaaaaagtgtttcatgtattactgaatctgatccatataagttcttaagaaaggaagataagtttgtacaagtttactttgaaaaaatacatcggtattacttcactattttttttgttttcaaatattctaattgctgaagagtttatttttgtagaaaaaaacttgagttttttccctaaattagggataattgtgcttgttttttttatgagtgctcccgcttttgttgttgttactttaattttgacttgtttagttgcatttcttattagtttaattaacaaattttacagtttcaaaagagtatacttatcgactttatttgtaaatagtattcagttattcgtaaatttagctttatttagtgtatttttacattacaatttaaatttgcgattgctaagtataatgagttttatgattaatatttttttagtagttatctatcgcaatttattaattaaatttgcgaatgtaaacagtagggctgcgaatgtattatcaattttcgggattgctttatctgtaatttatttggtggtaggagtaaagtaatgaaaaaaataacaattaacaacttgagtttttattatgaatccaaagatattatggtgtttgacaggttatctttagaatttt

SEQ ID NO: 4 - DNA, 15314 bp, Artificial Sequence
  synthetic
agtttctttttccgtgtgaatatcaaaatcaataaagaaggtattgatttgtcttaaattgttttcagaatgtcctttagtgtatgaacggttttcgtctgcatacgtaccataacgataaacgtttggtgtccaatgcgtaaatgtatcttgattttcgtgaatcgcttcttcggaagtcagaacaacgccacgtccgccaatcatgcttttttttgagcgatacgcaaaaatagcccctttacttttactggcttggtagtgattgagcgaattttactatttttaaatttgtactttaacaagccgtcatgaagcacagtttctacaacaaaagggatattcattcagctgttctcctttcttacgaaaattaattagttagaagctacgatcaaagttgaatcacaacaaaaaaggcaatcaactaagtttttcttaattgattgcctggtatcttcttaaagacttgaaatcccctcaaaaacccgatataatgggtttacagatatttaagtatctgattaataaagtaattaaatactttaccaaattttgggtctcgacttctttaattgattggtggtaatcaattaaggctcgcagttaaaatttctcaggctttaactggtcgtggctctttttttgtattctttattcagttcgttgtttcgttatatctagtatatcgctttttaaaaaaataagcaatgatttcgtgcattattcacacgaaatcattgcttttttcttcttccatttctaactccaatgttacttgttctgtttctggttctggttctgttggctcatttgggattaaatccactactagcgttgagttagttccgtctctaatagccggttaagtaatagccggttaagtggtcaaactttgggaaaatctcaacccgcattaagttttgatgccatgacaatcgttggaaatttgaacaaaactaatgctaaaaagctatctgactttatgagtgtagagccacaaatacgactttgggatatacttcaaacaaagtttaaagctaaggcacttcaagaaaaagtttatatcgaatatgacaaagtaaaagcagatacttgggatagacgtaatatgcgtgttgaatttaatcccaataaactcacacatgaagaaatgatttggttaaaacaaaatattatcgactacatggaagatgacggttttacaagattagacttagcttttgattttgaagatgatttgagcgattactatgcaatgactgataaagcagttaagaaaactgttttttatggtcgtaatggcaagccagaaacaaaatattttggtgtccgtgatagtgatagatttattagaatttataataaaaaacaagaacgtaaagataacgcagatgttgaagttgtgtttgaacatttatggcgtgtagaagttgaattaaaaagagatatggttgattactggaatgattgttttaatgatttacacatctttgaaacctgcgtgggctactttagaaaaaattaatgagcaagctatggtttatactttgttgcatgaagaaagtatgtggggaaagctaagtaagaatactaagactaaatttaaaaaattgattagagaaatatctccaattgatttaacggaattaatgaaatcgactttaaaagcgaacgaaaaacaattgcaaaagcagattgatttttggcaacgtgaatttaggttttggaagtaaaataagttttatttgataaaaattgctaattcagtataattaatatttacgaggtgacataacgtatgaaaaaatcagaggattattcctcctaaatataaaaatttaaaatttaggaggaagttatatatgacttttaatattattgaattagaaaattgggatagaaaagaatattttgaacactattttaatcagcaaactacttatagcattactaaagaaattgatattactttgtttaaagatatgataaaaaagaaaggatatgaaatttatccctctttaatttatgcaattatggaagttgtaaataaaaataaagtgtttagaacaggaattaatagtgagaataaattaggttattgggataagttaaatcctttgtatacagtttttaataagcaaactgaaaaatttactaacatttggactgaatctgataaaaacttcatttctttttataataattataaaaatgacttgcttgaatataaagataaagaagaaatgtttcctaaaaaaccgatacctgaaaacaccataccgatttcaatgattccttggattgattttagttcatttaatttaaatattggtaacaatagcagctttttattgcctattattacgataggtaaattttatagtgagaataataaaatttatataccagttgctctgcaacttcatcattctgtatgtgatggttaccatgcttcactatttatgaatgaatttcaagatataattcatagggtagatgattggatttagtttttagattttgaaagtgaatttaattttatacacgtaagtgatcataaaatttatgaacgtataacaaccacattttttggttgcttgtggttttgattttgaatttggttttgaacttatggactgatttattcagtccattttttgtgcttgcacaaaaactagcctcgcagagcacacgcattaatgacttatgaaacgtagtaaataagtctagtgtgttatactttacttggaagatgcaccgaataaaaaatattgaagaacaactagcaaaagattttaaagagttattttattttaagtctttataacatgagtgaagcgaatttttaaatttcgatagaaatttttacatcaaaaagccccctgtcaaaattgacgaagggggttttttggcgcacgcttttcgttagaaatatacaagattgaaaatcgtgtataagtgcgccctttgttttgaacttagcacgttacatcaattttttaaaatgatgtataagtgcgcccttttaaattttgagtgattatattttttgagttagaaaaagggattgggaaaatttcccaaaataatttaaaaaataagcaaaaattttcgatagagaatgtgctattttttgtcaaaggtgtataccttgactgtgcttgctgttacattaagtttatttttaagttattaaaaaagaaatagcttttaaagtttggctcgctgtcgctttataaagctgattgacttttgattgcaaactacttaaagaaaacaaactcggactattcgttttcttctctttggtttgaacatcagcaattatcccctcttgattgcctattttagcttgtttagaagaaacaaaagctaaaagctcctcttgggttttaaaacgctgtgtggggcttagaacgcccttaaacgacccttggtttacttttatactagcttccacctcgaaaaaaggttcttttttaaaattctctatggcttcctggcgctgaaaaaataaggtataaggtgggcgtttgaacacgtcctagtgaaaatgtaccttgtacgccccttctgttgtaaatttaacgtatacaaagggcttgcgttcatgccgatcaaccaatcggcaatttggcgtgtttgcgcttcttgataaaagggatagtaattcattccaggttgcaaattttgaaaaccgcttcggattacatctttttctaagctattgatccatagtcttttaaatgttttatcttttgaaaaggcatttgctttatggataatcgaccaggcgatattttcaccttctctgtcgctatctgttgcaacaataattgtatttgcctttttgagaagttctgcaacaattttaaactgctttcccttatcttttgcaacttcaaaatcgtatcgatcaggaaaaatcggcaaagattcaagtttccaattttgccacttttcgtcataatgacctggttctgctaattccactaaatgcccaaaaccaaaggtgataaacgtttcatctgtaaatagtgggtctttgatctcaaaataaccgtcttttttggtgctttgttttaaagcacttgcgtaggctaatgcctggcttggtttttcagctaaaataaccgtactcattaactatccctcttttcattgttttttctttgatcgactgtcacgttatatcttgctcgataccttctaaacgttcggcgattgattccagtttgttcttcaacttctttatcggataaaccattcaaaaacaaatcgaaagccgagatgcgccgcgtgcggctgctggagatggcggacgcgatggatatgttctgccaagggttggtttgcgcattcacagttctccgcaagaattgattggctccaattcttggagtggtgaatccgttagcgaggtgccgccggcttccattcaggtcgaggtggcccggctccatgcaccgcgacgcaacgcggggaggcagacaaggtatagggcggcgcctacaatccatgccaacccgttccatgtgctcgccgaggcggcataaatcgccgtgacgatcagcggtccagtgatcgaagttaggctggtaagagccgcgagcgatccttgaagctgtccctgatggtcgtcatctacctgcctggacagcatggcctgcaacgcgggcatcccgatgccgccggaagcgagaagaatcataatggggaaggccatccagcctcgcgtcgcgaacgccagcaagacgtagcccagcgcgtcggccgccatgccggcgataatggcctgcttctcgccgaaacgtttggtggcgggaccagtgacgaaggcttgagcgagggcgtgcaagattccgaataccgcaagcgacaggccgatcatcgtcgcgctccagcgaaagcggtcctcgccgaaaatgacccagagcgctgccggcacctgtcctacgagttgcatgataaagaagacagtcataagtgcggcgacgatagtcatgccccgcgcccaccggaaggagctgactgggttgaaggctctcaagggcatcggtcgacgctctcccttatgcgactcctgcattaggaagcagcccagtagtaggttgaggccgttgagcaccgccgccgcaaggaatggtgcatgcaaggagatggcgcccaacagtcccccggccacggggcctgccaccatacccacgccgaaacaagcgctcatgagcccgaagtggcgagcccgatcttccccatcggtgatgtcggcgatataggcgccagcaaccgcacctgtggcgccggtgatgccggccacgatgcgtccggcgtagagttccagagaatcggatggtattaattttaaagaacaatcagtattctgaaaaacaaataaatgttctcgatcagttacaaaagttagattttaagattgaggaattagaaagtaccttacagatagaagatgagaggttcaatctggaagaatatcaagaagccatgattgatgaaaattatctttatgatatagatatcgtagagaaaacaaagaagtagttcaagcgtataaccaggatagaatgaaagataagtcaaatgaaaatgaacaatttgaaggaattagtcatgatattgattgctaagaagtatctagtgacttttttcttgattgaaactcaagatagatatgttattgcttgcatcaaaataaactacatgggtataatagcaatgaaatgcatttcaaaaatattttgaggaggagtatcatggttaaagaaaataaattttctaagatttttattttaatggctttgagttttttggggttagccttgtttagtgcaagtcttcagtttttgccgattgcacatatggctaaagagttcggtataccagcagcagttgcaggaactgtacttaatgtagttgaagctggtggatgggtcactactattgtatcaaatcttactgctgtaggtagcggaggtctttccttactcgctgcagcaggaagagagtcaattaaagcataccttaagaaagaaattaagaaaaaaggaaaaagagcagttattgcttggtaatttaacaatatgataaaaaaacaggatattttctagagatattctgttttttaattaaaaaaaggggggcgctcatgaatctctttggaattctaatgaagttaagaataaatcaagagagtagtttggttaaaagagtactttcctactttaacttaaaactatcgttaaagctctatttatttattaatatattctttgaattttcattggcatttgttgttagtttgggattaagactaactttaataaaatcagatataaatgtaaatttattttttataatattttttattttaggaattgttcaaggagcatcaaattgttatagaacgcacgtctttccttttgaagaattaaggaaattagcaacaatatcttctagaaagataagctttattatgattgttacagacttattctatatttttatgttttcatcttcaatactatatggattattgagtttaatatatataagtagtaatgcttttatttttcaaaaaattagtctatctgtattttttttatttatatacatttgttcattttattgtagtaataggatttttggacagtatatctataataaaatagttaaggctattggattaacacgattaatcctttatagcattggagccgctttatttacttattttggtttttttatagtatcattcgtatttagtaacatagtatattttataaaaaaatattttgttaacatagaaagtgtaaataataaagtaatatgggagtcgttttctaaggatataggaatgttttatgtaaatagcgccagtaaattttatgagagtcatgtatattcatttacttatatagatgtttttttagtatcggctatgttattaattttggcaatattactattagctatggaaccaaaactctaccctttaaaaacaaaaatgctgccaaaaactaaaatagacttatgcaatttatatgtattttttttgaataaagcattaaaaaaaaatattttttttaaatgcagcttgttaaagttagctaatacaagatggattattgctaataatttctttcaaaatataattttgacatatgaatcattcttttacattggagtaatgctttcaataatactattgaattcacaaaatagaatgttgcaaatacaactattatttcttttaaatatacttgtaattggaaatcagacatttgaaataagagaagaaatgtacccttatctatcttttggatcagaaaggaatcaatttacgcttctaagatcgtctccgaatggtttgaataaagtttttaattcgaaactaacgatatacaggttatttttattaattcctttacttatattaattatcataaatattgtagtttctgtatacattatgattccggtaatttttgctatctttttgtttataacattttctatgtctgtgtatgttttccctatgattcaaatgtatatgattcctttagctactaaactagattacactaatgatacagaaattggaagtgctaaagatgaaaaaattgttttagagaaatttcaaacagttccaagatacttttttaatatcgttcctttagtgcttacatttatctttccaattgtaggggaaagttattcattaataatatttttcggagagttagtatatttctctttagcaacaataatatttgtgtttttcagtaaaaaaattattaggaaaggaatttttgttgtacatgcgattagatatcattaattttgagaaatatttgaaaatttccttctatatatcaatatttattttttttctgggagtgttagcagggattataataggtcctcatataaataaattggactattttggtcaggaagtttcattttatagtgttagtgttaataatttaaaggtctctttttatttcctcactataggaatggtaacaggggggatttatgcatttttatttatgggtataaatggttatataattggtaagttgattcaatatttatacattaacaatgaactaaatgttttgtataaaggtcttcttccacatttttttatagagcttttaggattggcaacatttagtatgataagtaccattccaatatttgttattttggttttttttaaaacgcctacacatgtagttcctattaaaaaaatcataaagttaagtgtgttttttactgtacttggaatagttttaataataattggaggatatatagaatctaatataagctatgtagatatacgatagaagttgagatagaaaactaatctcaaaggaagatatccgcctatttccaaacgttatacgaaagaatttaaacaaaccattgatcacgaatcaaaaatgctgaattaaagatatactcattaaaggaagagtgggcactattttaaatttatacaaccaaggtaaaaattttcgtgaattatctttataataatatgtcggttacttaaaatttttgaaattcacaataaacatataattaacagtgtgataatttatttgtctacaagtcaattgggataggcaactctagttgcataaaatatctctcacaaaaagtgtttcatgtattactgaatctgatccatataagttcttaagaaaggaagataagtttgtacaagtttactttgaaaaaatacatcggtattacttcactattttttttgttttcaaatattctaattgctgaagagtttatttttgtagaaaaaaacttgagttttttccctaaattagggataattgtgcttgttttttttatgagtgctcccgcttttgttgttgttactttaattttgacttgtttagttgcatttcttattagtttaattaacaaattttacagtttcaaaagagtatacttatcgactttatttgtaaatagtattcagttattcgtaaatttagctttatttagtgtatttttacattacaatttaaatttgcgattgctaagtataatgagttttatgattaatatttttttagtagttatctatcgcaatttattaattaaatttgcgaatgtaaacagtagggctgcgaatgtattatcaattttcgggattgctttatctgtaatttatttggtggtaggagtaaagtaatgaaaaaaataacaattaacaacttgagtttttattatgaatccaaagatattatggtgtttgacaggttatctttagaattttcttctgaaaaaagttatgcactagttggttctaatggtgtaggaaaaacaacattgttaaatattttatcaggtatatatcaacccacagggggaacaatagaatatgacagcactttgtatacagaaaaagtaactaaagaaaaagtagcttttataccatataaaactaagctatatccttatcttgatgtttttgatcatataaagctaatagcagaattatggggaattaaaacagactatttagaatataaaagaaaagtactagaatattgtagccgtctaaacttggactattataataagaaagtagagtcttactctacaggtatggagtataaactatacatttctttaatgttggcaagagatgtttctcttgtattattagatgaaccttttacaatgttagataaaaaaagtcgatatttagctatggacttaatcaaagagaaaaaaataataacaatattttcttcacatcagaaagatattgtagaatatttgtcaaatgatattattaatcttgacaaactgaagggagtaaacttggaaaattatgaaaagaattgattacattattattatagtctcactattagcaacaatagtcgcaatatttttaatagggatagattctatgttaggcacaggacgggtgtggtcgccatgatcgcgtagtcgatagtggctccaagtagcgaagcgagcaggactgggcggcggccaaagcggtcggacagtgctccgagaacgggtgcgcatagaaattgcatcaacgcatatagcgctagcagcacgccatagtgactggcgatgctgtcggaatggacgatatcccgcaagaggcccggcagtaccggcataaccaagcctatgcctacagcatccagggtgacggtgccgaggatgacgatgagcgcattgttagatttcatacacggtgcctgactgcgttagcaatttaactgtgataaactaccgcattaaagcttatcgatgataagctgtcaaacatgagaattacaacttatatcgtatggggctgacttcaggtgctacatttgaagagataaattgcactgaaatctagaaatattttatctgattaataagatgatcttcttgagatcgttttggtctgcgcgtaatctcttgctctgaaaacgaaaaaaccgccttgcagggcggtttttcgaaggttctctgagctaccaactctttgaaccgaggtaactggcttggaggagcgcagtcaccaaaacttgtcctttcagtttagccttaaccggcgcatgacttcaagactaactcctctaaatcaattaccagtggctgctgccagtggtgcttttgcatgtctttccgggttggactcaagacgatagttaccggataaggcgcagcggtcggactgaacggggggttcgtgcatacagtccagcttggagcgaactgcctacccggaactgagtgtcaggcgtggaatgagacaaacgcggccataacagcggaatgacaccggtaaaccgaaaggcaggaacaggagagcgcacgagggagccgccagggggaaacgcctggtatctttatagtcctgtcgggtttcgccaccactgatttgagcgtcagatttcgtgatgcttgtcaggggggcggagcctatggaaaaacggctttgccgcggccctctcacttccctgttaagtatcttcctggcatcttccaggaaatctccgccccgttcgtaagccatttccgctcgccgcagtcgaacgaccgagcgtagcgagtcagtgagcgaggaagcggaatatatcctgtatcacatattctgctgacgcaccggtgcagccttttttctcctgccacatgaagcacttcactgacaccctcatcagtgccaacatagtaagccagtatacactccgctagcgctgatgtccggcggtgcttttgccgttacgcaccaccccgtcagtagctgaacaggagggacagctgatagaaacagaagccactggagcacctcaaaaacaccatcatacactaaatcagtaagttggcagcatcacccgacgcactttgcgccgaataaatacctgtgacggaagatcacttcgcagaataaataaatcctggtgtccctgttgataccgggaagccctgggccaacttttggcgaaaatgagacgttgatcggcacgtaagaggttccaactttcaccataatgaaataagatcactaccgggcgtattttttgagttatcgagattttcaggagctaaggaagctaaaatggagaaaaaaatcactggatataccaccgttgatatatcccaatggcatcgtaaagaacattttgaggcatttcagtcagttgctcaatgtacctataaccagaccgttcagctggatattacggcctttttaaagaccgtaaagaaaaataagcacaagttttatccggcctttattcacattcttgcccgcctgatgaatgctcatccggaattccgtatggcaatgaaagacggtgagctggtgatatgggatagtgttcacccttgttacaccgttttccatgagcaaactgaaacgttttcatcgctctggagtgaataccacgacgatttccggcagtttctacacatatattcgcaagatgtggcgtgttacggtgaaaacctggcctatttccctaaagggtttattgagaatatgtttttcgtctcagccaatccctgggtgagtttcaccagttttgatttaaacgtggccaatatggacaacttcttcgcccccgttttcaccatgggcaaatattatacgcaaggcgacaaggtgctgatgccgctggcgattcaggttcatcatgccgtctgtgatggcttccatgtcggcagaatgcttaatgaattacaacagtactgcgatgagtggcagggcggggcgtaatttttttaaggcagttattggtgcccttaaacgcctggtgctacgcctgaataagtgataataagcggatgaatggcagaaattcgaaagcaaattcgacccggtcgtcggttcagggcagggtcgttaaatagccgcttatgtctattgctggtttaccggtttattgactaccggaagcagtgtgaccgtgtgcttctcaaatgcctgaggccagtttgctcaggctctccccgtggaggtaataattgacgatatgatcatttattctgcctcccagagcctgataaaaacggttagcgcttcgttaatacagatgtaggtgttccacagggtagccagcagcatcctgcgatgcagatccggaacataatggtgcagggcgcttgtttcggcgtgggtatggtggcaggccccgtggccgggggactgttgggcgctgccggcacctgtcctacgagttgcatgataaagaagacagtcataagtgcggcgacgatagtcatgccccgcgcccaccggaaggagctaccggacagcggtgcggactgttgtaactcagaataagaaatgaggccgctcatggcgttgactctcagtcatagtatcgtggtatcaccggttggttccactctctgttgcgggcaacttcagcagcacgtaggggacttccgcgtttccagactttacgaaacacggaaaccgaagaccattcatgttgttgctcaggtcgcagacgttttgcagcagcagtcgcttcacgttcgctcgcgtatcggtgattcattctgctaaccagtaaggcaaccccgccagcctagccgggtcctcaacgacaggagcacgatcatgcgcacccgtggccaggacccaacgctgcccgactttaaacgtggatcattttctttaaatttatgctgacgacctttgaatttgccttttttcttagcaatttcgattccttgtgcctgacgttccttaattttttttcgttctgattctgcttgatacttgtacaattcaatgacaaggctattaatcaaacgccttaaattttcatcttcaataccattcattgagggtaaatttaagacttccagggttgcccccttaatttgaatttgattcatcaattctgttaattctttattatttcgtcctaatcgatctaattcagtaacaataacaatatccccttcacgaatatagttaagcatagcttgtaattgtgggcgttcgaccgattgaccgcttaatttgtctgaaaagaccttagaaacgccctgtaacgcttgtaattgccgatctaagttctgttctttgctactgacacgtgcataaccaattttagccattttcaaccaacctctaaaattctctcggttgcaataaccaatcagcaatatctactttttcaatttcaaattgcttatcagaaattgtcttttcgtaagcgataaaatcttgcgcatattgttgctcattaaaaatagccaccacttcgtcattttctaaaactcgataaataaattttttcattttactcctcctattatgcccaacttaaatgacctattcaccaagtcaattatactgctaaaatcatattaggacaaataggtatactctattgacctataaatgatagcaacttaaaagatcaagtgttcgcttcgctctcactgcccctcgacgttttagtagcctttccctcacttcgttcagtccaagccaactaaaagttttcgggctactctctccttctccccctaataattaattaaaatcttactctgtatatttctgctaatcattcactaaacagcaaagaaaaacaaacacgtatcatagatataaatgtaatggcatagtgcgggttttattttcagcctgtatcgtagctaaacaaatcgagttgtgggtccgttttggggcgttctgccaatttgtttagagtttcttgaataaatgtacgttctaaattaaacgaagctgtcagcgcctttatatagctttctcgttcttctttttttaatttaatgatcgatagcaacaatgatttaacactagcaagttgaatgccaccatttcttcctggtttaatcttaaagaaaatttcctgattcgccttcagtaccttcagcaatttatctaatgtccgttcaggaatgcctagcacttctctaatctcttttttggtcgtcgctaaataaggcttgtatacatcgcttttttcgctaatataagccattaaatcttctttccattctgacaaatgaacacgttgacgttcgcttctttttttcttgaatttaaaccacccttgacggacaaataaatctttactggttaaatcacttgatacccaagctttgcaaagaatggtaatgtattccctattagccccttgatagttttctgaataggcacttctaacaattttgattacttctttttcttctaagggttgatctaatcgattattaaactcaaacatattatattcgcacgtttcgattgaatagcctgaactaaagtaggctaaagagagggtaaacataacgctattgcgccctactaaacccttttctcctgaaaatttcgtttcgtgcaataagagattaaaccagggttcatctacttgttttttgccttctgtaccgcttaaaaccgttagacttgaacgagtaaagcccttattatctgtttgtttgaaagaccaatcttgccattctttgaaagaataacggtaattgggatcaaaaaattctacattgtccgttcttggtatacgagcaatcccaaaatgattgcacgttagatcaactggcaaagactttccaaaatattctcggatattttgcgagattattttggctgctttgacagatttaaattctgattttgaagtcacatagactggcgtttctaaaacaaaatatgcttgataacctttatcagatttgataattaacgtaggcataaaacctaaatcaatagctgttgttaaaatatcgcttgctgaaat

SEQ ID NO: 5 - DNA, 10677 bp, Artificial Sequence
  synthetic
agtttctttttccgtgtgaatatcaaaatcaataaagaaggtattgatttgtcttaaattgttttcagaatgtcctttagtgtatgaacggttttcgtctgcatacgtaccataacgataaacgtttggtgtccaatgcgtaaatgtatcttgattttcgtgaatcgcttcttcggaagtcagaacaacgccacgtccgccaatcatgcttttttttgagcgatacgcaaaaatagcccctttacttttactggcttggtagtgattgagcgaattttactatttttaaatttgtactttaacaagccgtcatgaagcacagtttctacaacaaaagggatattcattcagctgttctcctttcttacgaaaattaattagttagaagctacgatcaaagttgaatcacaacaaaaaaggcaatcaactaagtttttcttaattgattgcctggtatcttcttaaagacttgaaatcccctcaaaaacccgatataatgggtttacagatatttaagtatctgattaataaagtaattaaatactttaccaaattttgggtctcgacttctttaattgattggtggtaatcaattaaggctcgcagttaaaatttctcaggctttaactggtcgtggctctttttttgtattctttattcagttcgttgtttcgttatatctagtatatcgctttttaaaaaaataagcaatgatttcgtgcattattcacacgaaatcattgcttttttcttcttccatttctaactccaatgttacttgttctgtttctggttctggttctgttggctcatttgggattaaatccactactagcgttgagttagttccgtctctaatagccggttaagtaatagccggttaagtggtcaaactttgggaaaatctcaacccgcattaagttttgatgccatgacaatcgttggaaatttgaacaaaactaatgctaaaaagctatctgactttatgagtgtagagccacaaatacgactttgggatatacttcaaacaaagtttaaagctaaggcacttcaagaaaaagtttatatcgaatatgacaaagtaaaagcagatacttgggatagacgtaatatgcgtgttgaatttaatcccaataaactcacacatgaagaaatgatttggttaaaacaaaatattatcgactacatggaagatgacggttttacaagattagacttagcttttgattttgaagatgatttgagcgattactatgcaatgactgataaagcagttaagaaaactgttttttatggtcgtaatggcaagccagaaacaaaatattttggtgtccgtgatagtgatagatttattagaatttataataaaaaacaagaacgtaaagataacgcagatgttgaagttgtgtttgaacatttatggcgtgtagaagttgaattaaaaagagatatggttgattactggaatgattgttttaatgatttacacatctttgaaacctgcgtgggctactttagaaaaaattaatgagcaagctatggtttatactttgttgcatgaagaaagtatgtggggaaagctaagtaagaatactaagactaaatttaaaaaattgattagagaaatatctccaattgatttaacggaattaatgaaatcgactttaaaagcgaacgaaaaacaattgcaaaagcagattgatttttggcaacgtgaatttaggttttggaagtaaaataagttttatttgataaaaattgctaattcagtataattaatatttacgaggtgacataacgtatgaaaaaatcagaggattattcctcctaaatataaaaatttaaaatttaggaggaagttatatatgacttttaatattattgaattagaaaattgggatagaaaagaatattttgaacactattttaatcagcaaactacttatagcattactaaagaaattgatattactttgtttaaagatatgataaaaaagaaaggatatgaaatttatccctctttaatttatgcaattatggaagttgtaaataaaaataaagtgtttagaacaggaattaatagtgagaataaattaggttattgggataagttaaatcctttgtatacagtttttaataagcaaactgaaaaatttactaacatttggactgaatctgataaaaacttcatttctttttataataattataaaaatgacttgcttgaatataaagataaagaagaaatgtttcctaaaaaaccgatacctgaaaacaccataccgatttcaatgattccttggattgattttagttcatttaatttaaatattggtaacaatagcagctttttattgcctattattacgataggtaaattttatagtgagaataataaaatttatataccagttgctctgcaacttcatcattctgtatgtgatggttaccatgcttcactatttatgaatgaatttcaagatataattcatagggtagatgattggatttagtttttagattttgaaagtgaatttaattttatacacgtaagtgatcataaaatttatgaacgtataacaaccacattttttggttgcttgtggttttgattttgaatttggttttgaacttatggactgatttattcagtccattttttgtgcttgcacaaaaactagcctcgcagagcacacgcattaatgacttatgaaacgtagtaaataagtctagtgtgttatactttacttggaagatgcaccgaataaaaaatattgaagaacaactagcaaaagattttaaagagttattttattttaagtctttataacatgagtgaagcgaatttttaaatttcgatagaaatttttacatcaaaaagccccctgtcaaaattgacgaagggggttttttggcgcacgcttttcgttagaaatatacaagattgaaaatcgtgtataagtgcgccctttgttttgaacttagcacgttacatcaattttttaaaatgatgtataagtgcgcccttttaaattttgagtgattatattttttgagttagaaaaagggattgggaaaatttcccaaaataatttaaaaaataagcaaaaattttcgatagagaatgtgctattttttgtcaaaggtgtataccttgactgtgcttgctgttacattaagtttatttttaagttattaaaaaagaaatagcttttaaagtttggctcgctgtcgctttataaagctgattgacttttgattgcaaactacttaaagaaaacaaactcggactattcgttttcttctctttggtttgaacatcagcaattatcccctcttgattgcctattttagcttgtttagaagaaacaaaagctaaaagctcctcttgggttttaaaacgctgtgtggggcttagaacgcccttaaacgacccttggtttacttttatactagcttccacctcgaaaaaaggttcttttttaaaattctctatggcttcctggcgctgaaaaaataaggtataaggtgggcgtttgaacacgtcctagtgaaaatgtaccttgtacgccccttctgttgtaaatttaacgtatacaaagggcttgcgttcatgccgatcaaccaatcggcaatttggcgtgtttgcgcttcttgataaaagggatagtaattcattccaggttgcaaattttgaaaaccgcttcggattacatctttttctaagctattgatccatagtcttttaaatgttttatcttttgaaaaggcatttgctttatggataatcgaccaggcgatattttcaccttctctgtcgctatctgttgcaacaataattgtatttgcctttttgagaagttctgcaacaattttaaactgctttcccttatcttttgcaacttcaaaatcgtatcgatcaggaaaaatcggcaaagattcaagtttccaattttgccacttttcgtcataatgacctggttctgctaattccactaaatgcccaaaaccaaaggtgataaacgtttcatctgtaaatagtgggtctttgatctcaaaataaccgtcttttttggtgctttgttttaaagcacttgcgtaggctaatgcctggcttggtttttcagctaaaataaccgtactcattaactatccctcttttcattgttttttctttgatcgactgtcacgttatatcttgctcgataccttctaaacgttcggcgattgattccagtttgttcttcaacttctttatcggataaaccattcaaaaacaaatcgaaagccgagatgcgccgcgtgcggctgctggagatggcggacgcgatggatatgttctgccaagggttggtttgcgcattcacagttctccgcaagaattgattggctccaattcttggagtggtgaatccgttagcgaggtgccgccggcttccattcaggtcgaggtggcccggctccatgcaccgcgacgcaacgcggggaggcagacaaggtatagggcggcgcctacaatccatgccaacccgttccatgtgctcgccgaggcggcataaatcgccgtgacgatcagcggtccagtgatcgaagttaggctggtaagagccgcgagcgatccttgaagctgtccctgatggtcgtcatctacctgcctggacagcatggcctgcaacgcgggcatcccgatgccgccggaagcgagaagaatcataatggggaaggccatccagcctcgcgtcgcgaacgccagcaagacgtagcccagcgcgtcggccgccatgccggcgataatggcctgcttctcgccgaaacgtttggtggcgggaccagtgacgaaggcttgagcgagggcgtgcaagattccgaataccgcaagcgacaggccgatcatcgtcgcgctccagcgaaagcggtcctcgccgaaaatgacccagagcgctgccggcacctgtcctacgagttgcatgataaagaagacagtcataagtgcggcgacgatagtcatgccccgcgcccaccggaaggagctgactgggttgaaggctctcaagggcatcggtcgacgctctcccttatgcgactcctgcattaggaagcagcccagtagtaggttgaggccgttgagcaccgccgccgcaaggaatggtgcatgcaaggagatggcgcccaacagtcccccggccacggggcctgccaccatacccacgccgaaacaagcgctcatgagcccgaagtggcgagcccgatcttccccatcggtgatgtcggcgatataggcgccagcaaccgcacctgtggcgccggtgatgccggccacgatgcgtccggcgtagagcacaggacgggtgtggtcgccatgatcgcgtagtcgatagtggctccaagtagcgaagcgagcaggactgggcggcggccaaagcggtcggacagtgctccgagaacgggtgcgcatagaaattgcatcaacgcatatagcgctagcagcacgccatagtgactggcgatgctgtcggaatggacgatatcccgcaagaggcccggcagtaccggcataaccaagcctatgcctacagcatccagggtgacggtgccgaggatgacgatgagcgcattgttagatttcatacacggtgcctgactgcgttagcaatttaactgtgataaactaccgcattaaagcttatcgatgataagctgtcaaacatgagaattacaacttatatcgtatggggctgacttcaggtgctacatttgaagagataaattgcactgaaatctagaaatattttatctgattaataagatgatcttcttgagatcgttttggtctgcgcgtaatctcttgctctgaaaacgaaaaaaccgccttgcagggcggtttttcgaaggttctctgagctaccaactctttgaaccgaggtaactggcttggaggagcgcagtcaccaaaacttgtcctttcagtttagccttaaccggcgcatgacttcaagactaactcctctaaatcaattaccagtggctgctgccagtggtgcttttgcatgtctttccgggttggactcaagacgatagttaccggataaggcgcagcggtcggactgaacggggggttcgtgcatacagtccagcttggagcgaactgcctacccggaactgagtgtcaggcgtggaatgagacaaacgcggccataacagcggaatgacaccggtaaaccgaaaggcaggaacaggagagcgcacgagggagccgccagggggaaacgcctggtatctttatagtcctgtcgggtttcgccaccactgatttgagcgtcagatttcgtgatgcttgtcaggggggcggagcctatggaaaaacggctttgccgcggccctctcacttccctgttaagtatcttcctggcatcttccaggaaatctccgccccgttcgtaagccatttccgctcgccgcagtcgaacgaccgagcgtagcgagtcagtgagcgaggaagcggaatatatcctgtatcacatattctgctgacgcaccggtgcagccttttttctcctgccacatgaagcacttcactgacaccctcatcagtgccaacatagtaagccagtatacactccgctagcgctgatgtccggcggtgcttttgccgttacgcaccaccccgtcagtagctgaacaggagggacagctgatagaaacagaagccactggagcacctcaaaaacaccatcatacactaaatcagtaagttggcagcatcacccgacgcactttgcgccgaataaatacctgtgacggaagatcacttcgcagaataaataaatcctggtgtccctgttgataccgggaagccctgggccaacttttggcgaaaatgagacgttgatcggcacgtaagaggttccaactttcaccataatgaaataagatcactaccgggcgtattttttgagttatcgagattttcaggagctaaggaagctaaaatggagaaaaaaatcactggatataccaccgttgatatatcccaatggcatcgtaaagaacattttgaggcatttcagtcagttgctcaatgtacctataaccagaccgttcagctggatattacggcctttttaaagaccgtaaagaaaaataagcacaagttttatccggcctttattcacattcttgcccgcctgatgaatgctcatccggaattccgtatggcaatgaaagacggtgagctggtgatatgggatagtgttcacccttgttacaccgttttccatgagcaaactgaaacgttttcatcgctctggagtgaataccacgacgatttccggcagtttctacacatatattcgcaagatgtggcgtgttacggtgaaaacctggcctatttccctaaagggtttattgagaatatgtttttcgtctcagccaatccctgggtgagtttcaccagttttgatttaaacgtggccaatatggacaacttcttcgcccccgttttcaccatgggcaaatattatacgcaaggcgacaaggtgctgatgccgctggcgattcaggttcatcatgccgtctgtgatggcttccatgtcggcagaatgcttaatgaattacaacagtactgcgatgagtggcagggcggggcgtaatttttttaaggcagttattggtgcccttaaacgcctggtgctacgcctgaataagtgataataagcggatgaatggcagaaattcgaaagcaaattcgacccggtcgtcggttcagggcagggtcgttaaatagccgcttatgtctattgctggtttaccggtttattgactaccggaagcagtgtgaccgtgtgcttctcaaatgcctgaggccagtttgctcaggctctccccgtggaggtaataattgacgatatgatcatttattctgcctcccagagcctgataaaaacggttagcgcttcgttaatacagatgtaggtgttccacagggtagccagcagcatcctgcgatgcagatccggaacataatggtgcagggcgcttgtttcggcgtgggtatggtggcaggccccgtggccgggggactgttgggcgctgccggcacctgtcctacgagttgcatgataaagaagacagtcataagtgcggcgacgatagtcatgccccgcgcccaccggaaggagctaccggacagcggtgcggactgttgtaactcagaataagaaatgaggccgctcatggcgttgactctcagtcatagtatcgtggtatcaccggttggttccactctctgttgcgggcaacttcagcagcacgtaggggacttccgcgtttccagactttacgaaacacggaaaccgaagaccattcatgttgttgctcaggtcgcagacgttttgcagcagcagtcgcttcacgttcgctcgcgtatcggtgattcattctgctaaccagtaaggcaaccccgccagcctagccgggtcctcaacgacaggagcacgatcatgcgcacccgtggccaggacccaacgctgcccgactttaaacgtggatcattttctttaaatttatgctgacgacctttgaatttgccttttttcttagcaatttcgattccttgtgcctgacgttccttaattttttttcgttctgattctgcttgatacttgtacaattcaatgacaaggctattaatcaaacgccttaaattttcatcttcaataccattcattgagggtaaatttaagacttccagggttgcccccttaatttgaatttgattcatcaattctgttaattctttattatttcgtcctaatcgatctaattcagtaacaataacaatatccccttcacgaatatagttaagcatagcttgtaattgtgggcgttcgaccgattgaccgcttaatttgtctgaaaagaccttagaaacgccctgtaacgcttgtaattgccgatctaagttctgttctttgctactgacacgtgcataaccaattttagccattttcaaccaacctctaaaattctctcggttgcaataaccaatcagcaatatctactttttcaatttcaaattgcttatcagaaattgtcttttcgtaagcgataaaatcttgcgcatattgttgctcattaaaaatagccaccacttcgtcattttctaaaactcgataaataaattttttcattttactcctcctattatgcccaacttaaatgacctattcaccaagtcaattatactgctaaaatcatattaggacaaataggtatactctattgacctataaatgatagcaacttaaaagatcaagtgttcgcttcgctctcactgcccctcgacgttttagtagcctttccctcacttcgttcagtccaagccaactaaaagttttcgggctactctctccttctccccctaataattaattaaaatcttactctgtatatttctgctaatcattcactaaacagcaaagaaaaacaaacacgtatcatagatataaatgtaatggcatagtgcgggttttattttcagcctgtatcgtagctaaacaaatcgagttgtgggtccgttttggggcgttctgccaatttgtttagagtttcttgaataaatgtacgttctaaattaaacgaagctgtcagcgcctttatatagctttctcgttcttctttttttaatttaatgatcgatagcaacaatgatttaacactagcaagttgaatgccaccatttcttcctggtttaatcttaaagaaaatttcctgattcgccttcagtaccttcagcaatttatctaatgtccgttcaggaatgcctagcacttctctaatctcttttttggtcgtcgctaaataaggcttgtatacatcgcttttttcgctaatataagccattaaatcttctttccattctgacaaatgaacacgttgacgttcgcttctttttttcttgaatttaaaccacccttgacggacaaataaatctttactggttaaatcacttgatacccaagctttgcaaagaatggtaatgtattccctattagccccttgatagttttctgaataggcacttctaacaattttgattacttctttttcttctaagggttgatctaatcgattattaaactcaaacatattatattcgcacgtttcgattgaatagcctgaactaaagtaggctaaagagagggtaaacataacgctattgcgccctactaaacccttttctcctgaaaatttcgtttcgtgcaataagagattaaaccagggttcatctacttgttttttgccttctgtaccgcttaaaaccgttagacttgaacgagtaaagcccttattatctgtttgtttgaaagaccaatcttgccattctttgaaagaataacggtaattgggatcaaaaaattctacattgtccgttcttggtatacgagcaatcccaaaatgattgcacgttagatcaactggcaaagactttccaaaatattctcggatattttgcgagattattttggctgctttgacagatttaaattctgattttgaagtcacatagactggcgtttctaaaacaaaatatgcttgataacctttatcagatttgataattaacgtaggcataaaacctaaatcaatagctgttgttaaaatatcgcttgctgaaat

SEQ ID NO: 6 - DNA, 4637 bp, Artificial Sequence
  synthetic
ttccagagaatcggatggtattaattttaaagaacaatcagtattctgaaaaacaaataaatgttctcgatcagttacaaaagttagattttaagattgaggaattagaaagtaccttacagatagaagatgagaggttcaatctggaagaatatcaagaagccatgattgatgaaaattatctttatgatatagatatcgtagagaaaacaaagaagtagttcaagcgtataaccaggatagaatgaaagataagtcaaatgaaaatgaacaatttgaaggaattagtcatgatattgattgctaagaagtatctagtgacttttttcttgattgaaactcaagatagatatgttattgcttgcatcaaaataaactacatgggtataatagcaatgaaatgcatttcaaaaatattttgaggaggagtatcatggttaaagaaaataaattttctaagatttttattttaatggctttgagttttttggggttagccttgtttagtgcaagtcttcagtttttgccgattgcacatatggctaaagagttcggtataccagcagcagttgcaggaactgtacttaatgtagttgaagctggtggatgggtcactactattgtatcaaatcttactgctgtaggtagcggaggtctttccttactcgctgcagcaggaagagagtcaattaaagcataccttaagaaagaaattaagaaaaaaggaaaaagagcagttattgcttggtaatttaacaatatgataaaaaaacaggatattttctagagatattctgttttttaattaaaaaaaggggggcgctcatgaatctctttggaattctaatgaagttaagaataaatcaagagagtagtttggttaaaagagtactttcctactttaacttaaaactatcgttaaagctctatttatttattaatatattctttgaattttcattggcatttgttgttagtttgggattaagactaactttaataaaatcagatataaatgtaaatttattttttataatattttttattttaggaattgttcaaggagcatcaaattgttatagaacgcacgtctttccttttgaagaattaaggaaattagcaacaatatcttctagaaagataagctttattatgattgttacagacttattctatatttttatgttttcatcttcaatactatatggattattgagtttaatatatataagtagtaatgcttttatttttcaaaaaattagtctatctgtattttttttatttatatacatttgttcattttattgtagtaataggatttttggacagtatatctataataaaatagttaaggctattggattaacacgattaatcctttatagcattggagccgctttatttacttattttggtttttttatagtatcattcgtatttagtaacatagtatattttataaaaaaatattttgttaacatagaaagtgtaaataataaagtaatatgggagtcgttttctaaggatataggaatgttttatgtaaatagcgccagtaaattttatgagagtcatgtatattcatttacttatatagatgtttttttagtatcggctatgttattaattttggcaatattactattagctatggaaccaaaactctaccctttaaaaacaaaaatgctgccaaaaactaaaatagacttatgcaatttatatgtattttttttgaataaagcattaaaaaaaaatattttttttaaatgcagcttgttaaagttagctaatacaagatggattattgctaataatttctttcaaaatataattttgacatatgaatcattcttttacattggagtaatgctttcaataatactattgaattcacaaaatagaatgttgcaaatacaactattatttcttttaaatatacttgtaattggaaatcagacatttgaaataagagaagaaatgtacccttatctatcttttggatcagaaaggaatcaatttacgcttctaagatcgtctccgaatggtttgaataaagtttttaattcgaaactaacgatatacaggttatttttattaattcctttacttatattaattatcataaatattgtagtttctgtatacattatgattccggtaatttttgctatctttttgtttataacattttctatgtctgtgtatgttttccctatgattcaaatgtatatgattcctttagctactaaactagattacactaatgatacagaaattggaagtgctaaagatgaaaaaattgttttagagaaatttcaaacagttccaagatacttttttaatatcgttcctttagtgcttacatttatctttccaattgtaggggaaagttattcattaataatatttttcggagagttagtatatttctctttagcaacaataatatttgtgtttttcagtaaaaaaattattaggaaaggaatttttgttgtacatgcgattagatatcattaattttgagaaatatttgaaaatttccttctatatatcaatatttattttttttctgggagtgttagcagggattataataggtcctcatataaataaattggactattttggtcaggaagtttcattttatagtgttagtgttaataatttaaaggtctctttttatttcctcactataggaatggtaacaggggggatttatgcatttttatttatgggtataaatggttatataattggtaagttgattcaatatttatacattaacaatgaactaaatgttttgtataaaggtcttcttccacatttttttatagagcttttaggattggcaacatttagtatgataagtaccattccaatatttgttattttggttttttttaaaacgcctacacatgtagttcctattaaaaaaatcataaagttaagtgtgttttttactgtacttggaatagttttaataataattggaggatatatagaatctaatataagctatgtagatatacgatagaagttgagatagaaaactaatctcaaaggaagatatccgcctatttccaaacgttatacgaaagaatttaaacaaaccattgatcacgaatcaaaaatgctgaattaaagatatactcattaaaggaagagtgggcactattttaaatttatacaaccaaggtaaaaattttcgtgaattatctttataataatatgtcggttacttaaaatttttgaaattcacaataaacatataattaacagtgtgataatttatttgtctacaagtcaattgggataggcaactctagttgcataaaatatctctcacaaaaagtgtttcatgtattactgaatctgatccatataagttcttaagaaaggaagataagtttgtacaagtttactttgaaaaaatacatcggtattacttcactattttttttgttttcaaatattctaattgctgaagagtttatttttgtagaaaaaaacttgagttttttccctaaattagggataattgtgcttgttttttttatgagtgctcccgcttttgttgttgttactttaattttgacttgtttagttgcatttcttattagtttaattaacaaattttacagtttcaaaagagtatacttatcgactttatttgtaaatagtattcagttattcgtaaatttagctttatttagtgtatttttacattacaatttaaatttgcgattgctaagtataatgagttttatgattaatatttttttagtagttatctatcgcaatttattaattaaatttgcgaatgtaaacagtagggctgcgaatgtattatcaattttcgggattgctttatctgtaatttatttggtggtaggagtaaagtaatgaaaaaaataacaattaacaacttgagtttttattatgaatccaaagatattatggtgtttgacaggttatctttagaattttcttctgaaaaaagttatgcactagttggttctaatggtgtaggaaaaacaacattgttaaatattttatcaggtatatatcaacccacagggggaacaatagaatatgacagcactttgtatacagaaaaagtaactaaagaaaaagtagcttttataccatataaaactaagctatatccttatcttgatgtttttgatcatataaagctaatagcagaattatggggaattaaaacagactatttagaatataaaagaaaagtactagaatattgtagccgtctaaacttggactattataataagaaagtagagtcttactctacaggtatggagtataaactatacatttctttaatgttggcaagagatgtttctcttgtattattagatgaaccttttacaatgttagataaaaaaagtcgatatttagctatggacttaatcaaagagaaaaaaataataacaatattttcttcacatcagaaagatattgtagaatatttgtcaaatgatattattaatcttgacaaactgaagggagtaaacttggaaaattatgaaaagaattgattacattattattatagtctcactattagcaacaatagtcgcaatatttttaatagggatagattctatgttagg

SEQ ID NO: 7 - DNA, 735 bp, Enterococcus faecalis
atgcgcccaaaagagaaaaaaagaggaaaaaattggttaatcaacagtttattagttttactatttatcattggcttggccttaatttttaacaatcagatacgcagttgggtggttcaacaaaatagccgctcgtacgccgttagcaagttgaaaccagccgatgtgaagaaaaatatggctcgtgaaacaacgtttgactttgattcagttgagtccttgagcacagaagcggtgatgaaagcccaatttgaaaacaaaaacttacctgtgattggtgccattgcgataccaagtgtcgaaattaatttgcccatttttaaaggattgtcaaatgtcgctttattaactggtgccgggaccatgaaagaagatcaagtcatggggaaaaacaattatgccttggctagtcatcgaacggaagatggcgtttccttattttcacctttagaaagaaccaaaaaagacgaactcatttatatcactgatttatctactgtttatacatacaaaataacttctgtagaaaaaatcgaaccaacccgtgttgagttaattgatgacgttcctggtcaaaatatgattaccttaattacctgtggcgatttacaagcaacgacgcgaattgctgttcaaggaacattagcagcaacgacgcctattaaagacgccaacgacgatatgttaaaggctttccaattggagcaaaaaaccttagccgattgggtggcttaa

SEQ ID NO: 8 - DNA, 681 bp, Artificial Sequence
  synthetic
ccaaaagagaaaaaaagaggaaaaaattggttaatcaacagtttattagttttactatttatcattggcttggccttaatttttaacaatcagatacgcagttgggtggttcaacaaaatagccgctcgtacgccgttagcaagttgaaaccagccgatgtgaagaaaaatatggctcgtgaaacaacgtttgactttgattcagttgagtccttgagcacagaagcggtgatgaaagcccaatttgaaaacaaaaacttacctgtgattggtgccattgcgataccaagtgtcgaaattaatttgcccatttttaaaggattgtcaaatgtcgctttattaactggtgccgggaccatgaaagaagatcaagtcatggggaaaaacaattatgccttggctagtcatcgaacggaagatggcgtttccttattttcacctttagaaagaaccaaaaaagacgaactcatttatatcactgatttatctactgtttatacatacaaaataacttctgtagaaaaaatcgaaccaacccgtgttgagttaattgatgacgttcctggtcaaaatatgattaccttaattacctgtggcgatttacaagcaacgacgcgaattgctgttcaaggaacattagcagcaacgacgcctattaaagacgccaacgacgatatgtta

SEQ ID NO: 9 - DNA, 54 bp, Artificial Sequence
  synthetic
atgcgcaaggctttccaattggagcaaaaaaccttagccgattgggtggcttaa

SEQ ID NO: 10 - DNA, 57732 bp, Enterococcus faecium strain CK135 plasmid pPD1
tgatttgacgaagcaatgcttttgtgacacccatttgaggaatttctctatatttcttccagatcattttcccatgttctaaaacctgaaccgctagataaaatcgctcgttttccaatacataacaatttcctgtctttgtatgtatccgatagaccttttgtaaaatcattgtacccgtcactttttgtttcattcttgaacaccagccctttctaaaatttagcgataaaaaccaaaaaacggggaacatatacatgaactgtatacgttccccgtgtactgcaaccatcattccaccatacaaaacaatttatttaaagtaatctttttcctagaccaataaaggagtttaaaaaggtctggaaattcacttaaaaaaatgttataatgtatgttgtaacttatgttgcagtgttcgagaaccgagtatagttcatgggatcagcatgaattatttaactatcctcttgggttggtagcccaaagatagtcggttcttatttttagttacttttttctagtttcatggtataattcgtatgttggacgaagtcatactactagtggtgtggcttttttttaagaaacaagagttaatattagtgcaaacaataatgcagctatatgttttttttgttgtttcattaaatttacctcacttagtaactattcattacagttactactatagcattaaagtttactcattacaagtatatgtattttaaaaaagacgtttccgggaaaaataattcattttttatttattttcttttttttgccgattttcgtcatattcagaatacatttataggagttgaatatatgcatttaaatgaattaatgaaaatacaaagaaaaagcgagaaattatctcaagctaagttttatgaaggtatttttcagcgtaattcagcaagcctttttgaaaaccataatgaacattttttaaaaattgctgatttgccaattcttgcagatagaagtaatttaacaatacctgaaataattagaacttgtaatgaagattttaaaagtgtttttgataaagatttagaaacatattattttgttctttcaaaaattcaacaaaatcctgattcagaatacaatcaagaactctactctctttatcaaaaatctatacatgaaaaatttacttcgttaaaatacatgaatttatatttacttataaaattgcaaacctctagtttgatttcagaaattattcctgtggataaacaagatttagctgatataaaaaagatgttttcatcaagcaaaagatttgtattgtatcactataaaattctttctaatctatgcactatattcccttactctgatcttcagacattgatagagcaactatttcctttacgtgaagatagtgacgagcagattaaagatacagcttgtttatccttgtctaatgcaattgctctaagtatatttacaaaggattacagttcttgctttatacttctaaatcactttgaaactttgttatcaaattacactagttataaatataaattaagtttcatagcttcaagaaatatgcttctatactttacttctggagatatagagcatattatgaaagtattctcgtatgttgaaatattgaaacaagtggaaagccctgaatatgttgagcaattccataaaaacttacaaacaatcatttctaaaagtgatgatgaaaaagcaaaacaaatatttggtgttcttgacgatgatggacaagtattagaccccaaaaattttgaccacaaaaaaatagattaacttaaaacccaaaaaataagacattaaaaatcttattttttgggttttcctatccttacagttaaaataaattcttaattatatctagtccacctatgatatttccaacagtaccaccaatacttgctaaaataaataccaaaaatattctcaataccctatttttatatattttttttattgatagcaaatcttcatccattgtttgaaaatcatgaactttaggttttctgatggtagcttctactattgcagaaaatacacctattgataccattggtagtaacgttgcaagtggagcaagtactaaagaagtaataaccgtcaatggattagcaagtgctaagacagtaaagagtgcagctacgccgccattccatataccccatcgaatgatttgatttatacctatatccattcctaaaacaaaagaataaatcaataaaccaataattattaaaggtataatactttctaaaaccctagttgaccaaagtttgggtggtaatccgtctaattcctcaatatttgcttttcgattttcctttatatttttctcaactccatttaagtgagcttgaccaataacaacaactattttttctccttcttcatttagaatttttgtagacatatataagtctctctcaattaagaaagattcccacaattcagggtatgtttgctgtaattgttcaaatataggttcaaaattttctgaattaagaagtttcttcatttcttctttagaatcttctgctccttctaaaactttaccaaaagcatgtgggaaaagagctttttttcttagaggtatcaaccgccaaaaacgtttaaatgtaacttgtgaatctctatcgactaaagctaatttagccccaattttttctgcactattcactgcttggaaaaattctgctcctggcacagaatcatttatttttgccaaatgtttttgaattaaactgtatattacacttgagatcaaaactattaattttttttgtttaattacttgaacaatatctgtatctgaccattcatcaggattcatatatttattgtaccttgttttatcccattctaaacaaacagtatctggactttccttttcaattacctcttttaccaattctgcactctctttagatatatgagaggttccaacaagtataatttctcgtttatctaaaaaaattctacgtactaattccatacttcctcctctaattttgtaccatcatttttttgtaatcatatctagctccaacagggtgaatcactaagttccttattgtatttttttgaagtcgagctattcccacttgaaacacgggtataacgcccgcatcatctatcactatcttttctgctttttttaattcctgccaacgtttagaggaagtgtctttaatcaactcatcgtagtttttattagaatatccaccgtgattcaatggactattggtttcaaagtttgctaaaaaactaatagggtctgcataatcagcttgccatccgcttagacttatcgcaaaatcttttttagtcaaacgttccataaatacattagcaggtactggtgtgatattaactttcaacccttctaagttttcttctaattgaccttgtaaaaattctcctgcttttttttcaaactctccgtcacctactaaaatatctagttctagtttttcagagacactatctttacttttgacagtttcccaataagttcttgcctgttttttgttatactctactaatttttcattggcaaaatccttttttgtttttggattataagccatcttttcaggcacaacaccaacagaaggaatagatccattatctaataatttttcgactaagctatctctatcaattggatagctaatcgcttttcggacatttttattttttaaaagtttattctctccagtttggttcatttctaaaaacatcgtattcgccattaacgttgttgaatattctttatcttttttgtattgtttcgcatattctcccgcaagtggcgcatcgtccagttgtccgtcattatacaaattaattcctgtattaatttctttgacaacttggaaattaattttatccatagagacatcttttttatcccagtactctttatttttagaaatcgtccacttatcagaagtgcctaccccctctaaaattgttaagttaaatgccccatttgttacaattgcttttttagaagtaccatagtctttcccgtactctttaattgctttctgctgtactggatagtaagcggttaaggataacagatcagtaaaataaggtgttggttcaactaattcaatttctaatgttttctcaccaatacttttcactgctaaagtatcttttacttgttttcctgaagcaatttctttggcattttttatagcagaaaacagttccacatttggagaagctgttttaggatctacaactctttgccacgcggccacaaaatcactagcagttatttgtgtaccatcagaccacttagcgccatctctaatcacaatggtataagttttgccattattcgatacttttggttgaccagctgcgatggctggttgcggttgatttttttcatctaatcgatacaacccctccatcacattggctaataaagttatactcgtttgatctacagcagttgctgggtctaaactttggacaggtgtccctgcagtcaaagtcgctacctgttctacttttttttcggttacatcttgtgaatcttttgtggcagtatttataccacaactggctaataccaaaggtaataacccaatacctaaaaaacaaaacttcttgtacttcttcatttttatcaacctccgtagtttaaatttgctaactaattctagcgatatacaaataaaataaccaattaatagctattatatttacaattttatcaaataaactttaatagggatacaaaatacagaatgaaatttatccaaacgaatgaatcaattacttattgttcaatccaattatgcaaagttatctcagaacctttagacttattcccattatttatattttctttttctaacgcacatgcaacaaataaattataaaacgacttgtagaataggccttttggactttttacagtagaatctgtcttaattttatgcatcacacgacgcaaacatttgtcaatttcttcttgataatcctctccaatcaaaacaatgttgtattctttttctactttggtttttgcacgtataattgttcctacttgttcatgggcttcttgaatagtatcagaaaaagcagcaataaattttaagctatctttgcttaggaaagtgttctcttgaacttctgaaaactgatcgagcaataattgttgctgcaagacttcttttttagtatctaatgtatctaatgtatctaaataagaagtatagaatagattgtctgcgattttcgcaattacaggattttcgttgatatcattgactttttctgtatttgcgattttcgcaattacaggattttcgttgatatcactgactttttctgtacttgcgattttcgcaattacaggattaacattgttttgttcctcattgattttgaaaacatcttctgaagtaacgttaggttttccgagatatagcaggttaggtgtagtttctatttttccattaattttctttactctaccttttttttgtttaagaagattaactgcttcaagctctttttttatttttgatacttttccttctctgcaatttagcagagtcattaattcagcaactgtgtagataaaataaacattgtcttcactatctacccaattatttttaacggaattatcaaaccgatcttttaaaagcatgtatgcaatttttgcatcattggataatgatttgtaaacttcatttgtgaaaaatacttttggcatttgatagtatttttctctgtaaatttctttagatttgtaaaattgaaaattttccattttaaagctcctttagaatgtaagtgttatcaatcgtccacgtattcttatcttgtaaactacaggaatacaattcgattgtaaagtaatattttaacgcaatatttacacaagtacacaaatacacaagtgcaaaaatgtatttgtgtaaatatctaattttgaatattatcaggttaaacaaaattatgtgtacatttacacatttgtaaaaatacacatagcggaagactttcattattgattatattactaattacacaaataaaaatgtgtaaatgtgtaaaaaaacattgattatttaaattgcctattgtataatttaagcatagatatttacacaaatgtaaatgtgtaaatttgaaaaattacacataaaaaaaggaggaactttcatgatagagcttatagtagaagagtttgaacaactagccaatctattagaagaaaggtgcagagtaattagtataggtaaccaaaaaggtggtgtaggtaaatcttcccttgttcgtttacttccgtctgtgttagctttttcaggtaaaaaagttttactcatagatatggaccctcaagcgaatacaactaaaagtatgttcgtaacccgaaaaaattattatgaagacgaagttgttgtatttaaaaaaacattaatggctggtatcgttgaaggtaatcttactgatctagttatcaacgttttacctaatttagattttattccatcttcatcagatttagaaagtttccctacgtttctgtctaaaaagtttggattagttgataaaacagaccctgatttttatgaagtgaaagacaaagcctatgaatatttcaattcattgattgaatcattaaaagacaattatgattatatattctttgatacgccgcctacggtttctgattatgttagagctgtatcatatgttagtgattatatactaattgcatttcaaactcagagcgacagtttagacggtgcaaaagaatttttagaagatactttaatacctttagtagaaaatacaagagcagagtttgaagttgtaggtattttgcctaatcaaatgactaagaacggtagtattgacacttcatcacttaatgatgcatatacaatttttggaaaggaaaatgtatttgagaatattttgccttttaaaaaaccaatacaaaacatccctagacatggcgttacattagaaggttattggaatagtaaaatgtacattgatacattaataccaattactaaagaacttgtcacaagaattagtttaatagaaggagattagaccatgactgaaaatagaaaaccatcactaataggaaatagaaataaaaatctttatcaggaaacacctagaccagaacaaccttacagtggagctgaaaccatacctaaggatatcttagctaatgagaggggaacaatacgtgtgcctcttgatcaaaaaatagaatttgatgcattgttagcgacttctgaatatcattatacttatgagttaatggctgaacttgtatatgaagcagtcaaaaacaagactaaggaagagaataaaaaatatcaagaaacgttagcaatgttacgagagaaagaattgaaaaaaatagagagaaagaaaatgaaaaaataaaaatattcacatgtgtacttttgtaaatttacacatgtgaatatttttattatgaatcaatatatagcaagtaataattagttaaaaaattacacaattgtaaatgtccacatttacaaaaatacacatatatatcaacgacagtaaaactccctaaataatatagctatctttcatcaataatttttttagttcgtctgtgatgttctaagtgtagcaaataatcgtcttgcagttttagaaggtctgaatagacctgatccatagtcttgctggccgacaaagaaagagaataaataaatgagataggaagtgtttcaatttttttgttgcgagtaatccaagaagaaacagttccttgagagaaagcatgtaattcacaaaattcttctacagtaatccctagttgcttgataatgtatgcgttgatagggtgtggatatacaaaggtttttctaggcatggtgggtaagtttcctttcttagattattaatgcgtttgcagtaatattgtactaaaaaacatgcaataagggaagggcgtatctgcttctttttggttgacctcctttaaaaatatgttatactaaaggtgcgaaacgacattaaatcgtacaaataacacaaaaagcaatcctacggcgaataggattgcttttttttacactagttgcgactcctagcgtgtgtgttgatagcagcttactttcggttatcgtcttcctcgtccaacacacgagaaatcatttccagaaccaatcctacaaagatcggtgcgataaccaacgacattaaatctttcacaaataacacacctccaatcgaggcgagctgccgtattaattatatcatagattgaaattctgccaattcaataataaaaccttcaacaatttatctagctgttctatgatcttttctaagcgtgtaaactcgtttacaccaggaacatttatacttgtttgagtcactcgtaactctgcttgctagacagccacagctgcattctacataagccacttggtggacgctgtctcctagaggaataatggtaccattataatcatatgccttcattacgaaacccccaatcgctaaaatactcatctaactttttctgctctttttttgacaaagtaggggagactaaaccttgaaaagggtttgaatttactctttcttcttgttttattctactagaatgacgatacatacacacaaagtcaacttcttctatactataggaatcttcaccaattattattttgttttcttccgcatatcctctaaaagttcctataactggtctaggaaaaggattggtttctgaagacacaagtaataaatataatggcttattttgtttgattgagcgagaaaaataagaagaaaattcttttctattttgcttcatttggttgtacctaagccaacagttccacctgcatggccaccaacaaggcttgctcgtgaaattgctgtggcgccttccatcagtgaagaagcatgtatcagtgctttaaacccaaatttctgacgaattttatcaataagaaaatacatatccgtttcatgaatttgctcctccggaacagaaaataaatccagctgtaaatttttgttccatacaagacggccataggatacccctaaatttcgtacgtcgacccctggtgcgtaattctcttcaaaaagacgcagtacatgttcagtcaagacttttgtattattacttggttctactttcatttgtctacgccagccgttttggccgtatttgtctgtctgaccttttgagtagccaacaaacaaagagacacaggttgtctgacacgatgccatgcgtaagcgactagcgacctggtccgacaattccttcaaaaccaattttatttgttctttatttgcataatctttgggtaaaacctgactattgccaaatgatttttctgttggccgtcccgctttttgccctaaaaaactacgatctatgccccatgagtgcgcgtacagctgtagccccatgataccaaaacgctcttttaacatgtaaggttcaatgtgcgctaggtcataaatggaccgaatacctagcttttttaagcgagcagccatgcgatttcctatcccacaaaattctgtaagaggggagattggccaaactttttttggcacatcttcatagcgccattcagccacaaagcctggtgcattctttgcttcattatccaatgctaacttggccagcaacggattttccccaattccgattgtcacatacaatcccatatggttataaatcacacgttgaataatcttggccagtttataggcggtgtcacacttaaaataggtcagcgaagcagtcacatcaagaaacgattcatcgacactgaatacagaatgatcttcatcagaaacaaagcgtttatataaattgttaatttcttgatttttcttcatgtataatttcatgcgtggagatacaataattaagttcgggtggtccggaacttcatttttccttgtaacattggaaatgcctaatactttttttgccataggggaagcagcgagtaccaagccacccgaattttcagaattgctcatgaccacaagcattgtcttcaatggatcaagtccacgttctacgcattccacgctggcataaaaactttttacgtcgatacaaagcacatcacgactgggttctttcgtataatcgaacgtcaaattcatccaaaatcccttctttctactaacccattatacgaactaatgttctctttagcaactagtaaaattcagttttccgtatttttttacacctgtaaacttttggcatagttggactgaacgcagagagggaaactatacaaaacgttgaaggccagttgagcaaagcgaaaccaattattcgtcttttatattccagctgtattcctggaacaaataattattcgtatttaaaagggatttttcccattatttccgtctgcagtctatcatttaacaatataaatacgaacgttcaatatattctttgcataactaccgatcaatatttttgaaaacggcttagaattgctctctcatcactataattatcattaataattgaatatagaataacccccaaaaaaagattttcaggggtggggttttatttacttactaattttatcgatgcaagctttcccagtttcatcaagcaatggtgtaattcctcctttaggagtttctaaataattcacaccagtaacagtatcaactacaattttatagcctaatagagttaaagattcactttctttttcaacaaaacgtttgtctttaaatacatgttccttacatttatgtctgtctaatggtacgttatctgattgttctatcaactcactatttgaattatccccggcaaccatcatgcctaaatttttatcataataaatatattctccacctagtattaaggttaatggcataaaaatcttcctttctttaattttcttaccgtcctttttgttcattttctacgcacaatcaatcgattaaacagattgcctcttattccaacaagtaaatttcaagtgcaaatcatcctatttttaaataggatctgttgtcaactttttcttaattctatcaaaaaccggaagattttgcttgcaaaccaattcccttttactaaattaaaacaggtttttatttagtatgaaacagaaaccaacattgaagtaaatctcattatccattaaatttattgcaaagaccactaaaatatttaaaaaataactatgatttcattcttattgatacaccgcctgcaatgggaatgatttcggcaaacgtttttaattctgttgacgatgttttaattccatatcatcctgaagtatattctttcagaagtatggttaagtcaataaaatcaattaacaattttaaaagaagtaacaaaaatttaaatataaaagcagtgattccagttaaaataagaaaagtcctgactcacgaggcatttttacagtctgcacaagcattgtgtgaacaaaatagtatattaatgactaatacaacaattccagaatcaataagatatgcggaatctataggaaaatataaattacctgtcacacttattgatgaaaagaataaatccttaataggatacaaacaaatttatgcaaaattagcaagggagttgacctatattggctagaactaagaaaatagatggcttttcattcgaagatatcgtcaacactaatatcaataacgatattaatgataatgttaatgtcaatgataatggtaatgttaataatgatgttgatgataatttaaaagacaaggaaaatttcttggaaaatttaaaacctgaaaaagagaaaaaaattaaaacattactctatattgattctgatattgccaatcatttggacttctatggcgagaaactcggaaaaaaaatggtggtaaaagtaaattttgtaatgaattatttaaaaaatttttagaagataatagtttatggtcggaaaaaattgcttctaaaaaaagaaaataaaacaatagccataaatgcacatatatttatacgtatgtgtgtttcatggctattgtttttatttcaggaacttaagtgaaaagtaacaaccagttatgacggccagccgtcaaccatgacatcaactaatttattagcgtacgctacaataaattgagcattttcttctgtctcaatgggcacaagtgtgtcgccaataaattcatagagtggttgagaaataatttctttcattaagtctgtaggtaaaggaatcagccctggggttttatccatcagtcttttttcttcctcataaaaggcggtcattaaagaaagctcatctgtaacgggatctaagcagccataactacaagacaacatccggtccacaaccacagcttcaggcaaacctagtctcaaagcgatatacgctctaacaaaatatttttgatggatacttgccaacattgggcaggcatcctgccagtccaacacgatactctgttcctcatcttcttcatccatgaggcctagtaatacttctatgcccgattctaattcgtctttttcaaaaatacgctcaatagtcattgcttttaatcgtggaatagaagctaatatgttttcaattaatgcttcccaacgaacaagtttttctttaaagcgttttacttgggcttgttgttctaaagaaagagacgtttgttcccagaatgaaatttggtctttataagctgggacaagctctttttcagataagtacaagcgctctgttcttaagactgtctgatcatctaattgatagggaaccttaagagctggctgtaaagaatcgtagagctcttcagcagattctagttgacttgatagtagttgattcatcaggggaaaataatcaatcgtgtataaattttgattttctgtcatttgtttctccaattcttggaaatattttttaagactttattagaactgcccatgttcttctttgatttcaacgtactgtcctaggttcattttgtatttccgatgacaggttggacactcatagtaatttttttgataaacattctttgctagctccccgcaatcacattccacataaaaagcgatatttcgattaaaactagctatttcaataccccaacgatcataagattttcgcttcataaaaattttcctccttgtacattttactaacgattataaataccgttgccattctttcaactgttgactaattaacgcataaaattcgacttctgataaaatggtaatctcatgacctaacgcaatcaagtcccgcgcggtttgttccttttttgtatagagagaatcatcaaacaacgacttagaatactgaccacaaaccaggaaatttgtttttgaagtaacacttgattgacaatggccgtttaaagagtgaaccaaaccgatggcttgggttcgtgtcatttgctgcagcgttccagtaaaaacgaccctttgatccgttaagtccattttcaaactctcccttcccgtctaatagctgctatatctatcaagaaaagtggtgcaaggtattttcatattctttcactcgtcgataaaaggtatttcgtttcacgcccaattgctccatagcatagactgcagttatctttcctgctttccagtcagaatagatcgcaggaaattcaggaggtaaagcaattttctttctgccgaattttacaccctttcgtttcgcagcttctacgccttctctttgccggctattaattcgtttccgttcgtcttcggccatatagctcagtaattgcagaattaagtcagagataagcgtctctaatccatctagttgcttgtaactagcagtatctaacagaggcatgtctaacacagaaatatcaatctgcttttccttagttaattcccgccattcttctaaaatcatttgtttatttctgcctagtcgatctaatgattgtagatagagtaaatctccctttcgaaacattcgtttcattaattgatattcagggcgtttaaaatctttgccgctggctttttcaataaaaatatattcttcagggattcctaattctttcgcagcaattagttgtcgttcgatcgattgatcataactactgacccggatataaaaaaattttctcatcattattatctacccttttttcactaaaatcgtttcaaaaaacttacattaaatcagaaacgtttcaaattgtattatgtgattattatgccatatataaacaaagaaaatcaaggcatttcaaaaagtatactttttgaaacagatgaaaaaaatcagaggaacaaacaattattttgcctgttcctctgatttttattcatttcacttataaataagattaattttcgctaagcattcttcgattacttcttcaggggcttcctcaacgaaatcaaaacctcttgaaacaatatcaatacttctatgatgttcgagcaatatttcgcctgttattttcatatttttagtaagaggtacatgcagaggaaacgattttattttacttgtgataggcgcaacagataccatatttttaagatatgggaggcgctttcctagaataatacatgggcgctttccctgctgttcgtgtcctttagttggatttaaattaatatacacaacatcgccttgctttaattcatttacactttttttcataataactcttctcctacaggactgccccaatcatactctgtttcatttaaatctccacctttataatctgaaaataattcttctagcgtattaggaaatgtcgttttgggtgtaaggataatttgaccttgtctaataaccatttcaaatttggctgtttggccctttatacctagctctgctaattcttctttagataatcgaattcccttagaattaccccacttttttagctcaatttctttaactaacatatgatcacctcttctcgtccattataccacaaaaggatatacaagtatatacatttatgttttttctttttgcaacattccaacagtactttcattatcctattatgaaacgttagacttgcatgtttttaactttcacgacattattatcggtaagtttagtcattaattctttattcaaaaaagattgtgaactttttaggtagtagaattcttatattagtgcttctaattttttacgtataaaatttgaacttgaccatccataaatatatttttaagcagttaaaatccttaaaaaaagcagacctcaaggcctgcttttgaagaaactatttatccaatttttcttttacatctccaacaacatcttcgactttgtctttcgcatcagaagcgacttcttttactttaccaatagcttgatctaagaaaccttctgctttttgttgatcatcgccagtcacatttcctgccacttcttttgcttttcctttgattttatctgtcgttcctttatctgtcataatgaattcctcctgatattttatttttttagttgtttgtatctgaagactctaattctttactagcaccttcaatggctttactagcttttgtttttccttcttctactttttctttgcctttttcaactgcttcattggctttatctttcgcttcatcaagcgcgctgcttcctttttcctttgcctcttctactttagaagaagtagctgtagaattctctgttttcttttctttacttccgccacacgcagctaatgagaatacagctactccggcagcaattgtcaatacaatctttttcaactttcttcgacctccgtatatcaattttttatggtacatattaattataaaacaaatacatcaaaaaatataatggtctaaagtctgattttttatcttaaacactaaaaaagtgttgtgttggaaagttctcaaaaacaaaagtcaagtccaatttttatcctttaccttaatatatcgattaaatctttttttgctgcttctgatgcaggcattacagagaaaactagaccaataactgaagagacgccaactgctaataaaatagtaaatagatcaactgatacgtggacctttatcaaggagccaatgccataagcaaaaatcattcctaataaatagccaattatccctccagaaatagttaaaattaacccttctaaaaggaattgtaacataatcgattttcgagtagctcctaatgctcttcttataccaatttcttttgttcgctcagatacagagatatacatcatattcatgacccctacccctgcaataaacaatgatattcctgctacagctgttataaaataagtaattgtactgagaatctgaccaattcctttcgtcaacattgctgtatctaatacttcatattctcctagatgtcttaaactccctttctcttttaattgttttattactttagacgtcactttatcgggtttaactccttcttctaaagttaatgttaaagaggaggtatttttttccgatttaaaataatagcgatacgcatcttttggaatttcaatatttgtatttgacaaggaaaacaaattatcttgctcttctccaggaaaaactcctaccactctaaataattcttgctcaatttcaattcctttacccaatgctcgttctgatgtattaaatagctctttggctgtaactgaatcaattgttgctactttatttaataattcactatcttgacctgttaaattcctgccaatagaaactttttttccttcagaatctataagtttaatctgtttattttttttatttcctctaatagacaaatctttgtagatttgctcttcatcaattttagaatagtcagctttttttaccccttctacatttctcactgtagataagtctacatcttgaaagaattttgtatttgtatcatataaggacgtatcactcggtgtaaaatttaattgaatttccacatttttagaatcactcttagtaagattttttacggtatctttctcgaaccctcttccaatagctaaaattgtaataacagacgatattcctataataattcctatcatggttaatacactacgttttcgattatttttaattgctttccaagcagaacgcatgtttacataaagattcattgcaccaactccttatcttcaataatcgcaccgtctctaatagtaatcaaccggtgacaataaggaacgacttcagggttgtgcgtaaccataataagcgttacgtcatcttctttatttaaagtagtaaaaagcttcataatctcctctgaggtgtgtgtatctaaagcacctgtcggttcatctgctataataaacttagggtgattaatcaatgctcgggcaatggccacccgctgctgttggccaccagacaactgctttgggtatttatattcttttccttttaaaccaactctatccaatacggaaaaaactttttccttcgttttaaaaggagacaacccattataaagaagaggtagttctacattttcataaactgtgttactctcaatcaaactaaagttttggaaaataaaacctactgtttgatttcttattttagaaagaatgtcatctgctgtattaaccaaagatctgccttcaaacaagtattctccctcaaacttacgatcgataaatcccaaaagattaattaatgtcgatttgccagatcctgaagggcccatgatcgctatcatttccccttttttgatggataaatgaatatcttttaatacatgaagtgactcctcttcatttgcatagtatttatttatcttattgagttcaatcattgtttcaccgtcactttttggccatctttcagactagtatctgggttttcaatgattgaatcattttctttaagtccagtctttactacgtatttatcattatcttcttttacttctattttctgtttaacgacttttccatctctataaataaaaacgaatacctcattattattttctttaactgtattctttttagccaactctaaattattcattggaacactgatttggacattataaccataatgaataggttctttagggctaattataaaggagaatgttgaaattgtactatttttagttgatgatgtattttgtggactggcagccatatcttcaggcagtgcgttaatttcagtaattattccgtctgttgctttttcttcattgatttgactaatcgttacaggttgacccacttttactttattataatcatattctgtgacagaaccttttataactgtctctggactcacaatagtcgcatatggtactgttgcatctactttccctttatcgttaatatagacaattcctttgaatggtgctgttacggtagtggtaattttcttttttgtttgttcaatagtattattggcactggataaatcaacattcgccgcatctaacgcttgttgtgcttgtaaaactgcctctttttgtgcatctaacgcttgttgtatagtttcaattttattatcagcttcagctttttcggcttttttcatttcatcatccatttttttatttataatggtggtttgttcatttttagcaacagttaagcgattttctaattcttgttgtttttgtgttgcattatctaaatttatttgagcatttgtaactgctagattcaacttttctagagattgggtttgttcttccgcttgatcttcaacagttgtattttgataagtagcaactacatcattttcattgatttcttgaccattcttcacggaaatagtattaattttcccaagggattgatcaaaatttaaataattagttgttttaggttgaacaattccttttaaaaccaagggatcactcttttttaccttgataattttataggattcttcttcttttggttcactggcgttcaacttataaataatggtcgcgccaattaatagaactccaactatacagcctataatcgttaaagaaatttgttgttttttagttaactttttcaatatcattctcccctgtatttactttgaataggtaaactaaaaccataattaccggcagcttgaacactaatgtgaaaataatagttgtaattccgataattagtcctatagattgcgtttctgaagtatttgtaaaactaggcgttgttaacaaagaaaatataatggacacgacagtccatcccaaatttaaataatacggatattttagtggaatctgatctttttttatctttctatgtgaaataaaaaataaaatcacaaaagcaattgaaaaaataacatttaaaactgtgaacacttttactggcatactatttaattgattataaatatccatcccatcagatcctatgcttgtataaatcttttcgtttggatttaatgcactaggcaggccaataattgaaaaaattgttccgattgaaaccaacactagagcgattaaattccatattttaatcttttttacttcttttttataatcattcataacttcaaatcctctcttgtcataattaaagaatcctatctaaaaaaataaattttaactaagcttcctaagatttcataattcatatggtttcctctagtagatattgttacataaataaaattatttacataccccctttgccgatcagtctataaaaatcaacaaaaagtagtgtaattctattgtacagcttcttattttttaatttttatttattaatttatttatccattttaagaatggggaagaaaaaaatccgagagaaatagctaaaaaaatctttcctaacatagaatctatccctattaaaaatattgcgactattgttgctaatagtgagactataataataatgtaatcaattcttttcataattttccaagtttactcccttcagtttgtcaagattaataatatcatttgacaaatattctacaatatctttctgatgtgaagaaaatattgttattatttttttctctttgattaagtccatagctaaatatcgactttttttatctaacattgtaaaaggttcatctaataatacaagagaaacatctcttgccaacattaaagaaatgtatagtttatactccatacctgtagagtaagactctactttcttattataatagtccaagtttagacggctacaatattctagtacttttcttttatattctaaatagtctgttttaattccccataattctgctattagctttatatgatcaaaaacatcaagataaggatatagcttagttttatatggtataaaagctactttttctttagttactttttctgtatacaaagtgctgtcatattctattgttccccctgtgggttgatatatacctgataaaatatttaacaatgttgtttttcctacaccattagaaccaactagtgcataacttttttcagaagaaaattctaaagataacctgtcaaacaccataatatctttggattcataataaaaactcaagttgttaattgttatttttttcattactttactcctaccactaaataaattacagataaagcaatcccgaaaattgataatacattcgcagccctactgtttacattcgcaaatttaattaataaattgcgatagataactactaaaaaaatattaatcataaaactcattatacttagcaatcgcaaatttaaattgtaatgtaaaaatacactaaataaagctaaatttacgaataactgaatactatttacaaataaagtcgataagtatactcttttgaaactgtaaaatttgttaattaaactaataagaaatgcaactaaacaagtcaaaattaaagtaacaacaacaaaagcgggagcactcataaaaaaaacaagcacaattatccctaatttagggaaaaaactcaagtttttttctacaaaaataaactcttcagcaattagaatatttgaaaacaaaaaaaatagtgaagtaataccgatgtattttttcaaagtaaacttgtacaaacttatcttcctttcttaagaacttatatggatcagattcagtaatacatgaaacactttttgtgagagatattttatgcaactagagttgcctatcccaattgacttgtagacaaataaattatcacactgttaattatatgtttattgtgaatttcaaaaattttaagtaaccgacatattattataaagataattcacgaaaatttttaccttggttgtataaatttaaaatagtgcccactcttcctttaatgagtatatctttaattcagcatttttgattcgtgatcaatggtttgtttaaattctttcgtataacgtttggaaataggcggatatcttcctttgagattagttttctatctcaacttctatcgtatatctacatagcttatattagattctatatatcctccaattattattaaaactattccaagtacagtaaaaaacacacttaactttatgatttttttaataggaactacatgtgtaggcgttttaaaaaaaaccaaaataacaaatattggaatggtacttatcatactaaatgttgccaatcctaaaagctctataaaaaaatgtggaagaagacctttatacaaaacatttagttcattgttaatgtataaatattgaatcaacttaccaattatataaccatttatacccataaataaaaatgcataaatcccccctgttaccattcctatagtgaggaaataaaaagaaacctttaaattattaacactaacactataaaatgaaacttcctgaccaaaatagtccaatttatttatatgaggacctattataatccctgctaacactcccagaaaaaaaataaatattgatatatagaaggaaattttcaaatatttctcaaaattaatgatatctaatcgcatgtacaacaaaaattcctttcctaataatttttttactgaaaaacacaaatattattgttgctaaagagaaatatactaactctccgaaaaatattattaatgaataactttcccctacaattggaaagataaatgtaagcactaaaggaacgatattaaaaaagtatcttggaactgtttgaaatttctctaaaacaattttttcatctttagcacttccaatttctgtatcattagtgtaatctagtttagtagctaaaggaatcatatacatttgaatcatagggaaaacatacacagacatagaaaatgttataaacaaaaagatagcaaaaattaccggaatcataatgtatacagaaactacaatatttatgataattaatataagtaaaggaattaataaaaataacctgtatatcgttagtttcgaattaaaaactttattcaaaccattcggagacgatcttagaagcgtaaattgattcctttctgatccaaaagatagataagggtacatttcttctcttatttcaaatgtctgatttccaattacaagtatatttaaaagaaataatagttgtatttgcaacattctattttgtgaattcaatagtattattgaaagcattactccaatgtaaaagaatgattcatatgtcaaaattatattttgaaagaaattattagcaataatccatcttgtattagctaactttaacaagctgcatttaaaaaaaatatttttttttaatgctttattcaaaaaaaatacatataaattgcataagtctattttagtttttggcagcatttttgtttttaaagggtagagttttggttccatagctaatagtaatattgccaaaattaataacatagccgatactaaaaaaacatctatataagtaaatgaatatacatgactctcataaaatttactggcgctatttacataaaacattcctatatccttagaaaacgactcccatattactttattatttacactttctatgttaacaaaatatttttttataaaatatactatgttactaaatacgaatgatactataaaaaaaccaaaataagtaaataaagcggctccaatgctataaaagattaatcgtgttaatccaatagccttaactattttattatagatatactgtccaaaaatcctattactacaataaaatgaacaaatgtatataaataaaaaaaatacagatagactaattttttgaaaaataaaagcattactacttatatatattaaactcaataatccatatagtattgaagatgaaaacataaaaatatagaataagtctgtaacaatcataataaagcttatctttctagaagatattgttgctaattttcttaattcttcaaaaggaaagacgtgcgttctataacaatttgatgctccttgaacaattcctaaaataaaaaatattataaaaaataaatttacatttatatctgattttattaaagttagtcttaatcccaaactaacaacaaatgccaatgaaaattcaaagaatatattaataaataaatagagctttaacgatagttttaagttaaagtaggaaagtactcttttaaccaaactactctcttgatttattcttaacttcattagaattccaaagagattcatgagcgcccccctttttttaattaaaaaacagaatatctctagaaaatatcctgtttttttatcatattgttaaattaccaagcaataactgctctttttccttttttcttaatttctttcttaaggtatgctttaattgactctcttcctgctgcagcgagtaaggaaagacctccgctacctacagcagtaagaattgatacaatagtagtgacccatccaccagcttcaactacattaagtacagttcctgcaactgctgctggtataccgaactctttagccatatgtgcaatcggcaaaaactgaagacttgcactaaacaaggctaaccccaaaaaactcaaagccattaaaataaaaatcttagaaaatttattttctttaaccatgatactcctcctcaaaatatttttgaaatgcatttcattgctattatacccatgtagtttattttgatgcaagcaataacatatctatcttgagtttcaatcaagaaaaaagtcactagatacttcttagcaatcaatatcatgactaattccttcaaattgttcattttcatttgacttatctttcattctatcctggttatacgcttgaactacttctttgttttcttctacgatatctatatcataaagataattttcatcaatcatggcttcttgatattcttccagattgaacctctcatcttctatctgtaaggtactttctaattcctcaatcttaaaatctaacttttgtaactgatcgagaacatttatttgtttttcagaatactgattgttctttaaaattaataccatccgattctctggaacaacctgaatcatttcttccatcgtcatggaccaaaaatcagggtgataacggtcaatagacggatctttaaaaaacgcttcaattgttccgtggtcaacatctcgaatacgaccatcgccaccctcagaataaccactccataaagaaccatctttaaaaacataaatggcttgttctaaattgtctgttttttcgaatccttcgtcaataaaatcagaaaaatcaaatcttgaactcgtttctttcatcacgttttccccatttcttctttttattatttggtaaacaaaaagagcataacgggtggttatgctcttttttttacgtcttaaattgtttgagaattatttatttttaaatagacatgctttgttctagttcctggtaaactttttcattcaagtatcgctgcaagcttccctgacaagctttacgtaaatgacgcatctgttttctaaattgtacatccgaatatttctgtggattttgcttaattgacactggtttttttctcattgtgccacgtcgttgctcaattttacgatcaacattgcgaactttttctggcagttcttctgtttgagaaatatcaaaaatttcttttttctcaaacgtaaacgacccatctgcttctttttttagagacacaatttctattgggttgtctttttcttcttcttttacttgacgattattgagttgccattgcttatcgcctaagagaaacgtcgcttgtggattggtttgtaagatagctcgttgattgccatttgaaaacacatgtaaattcgtttttattttcttgttgttttcgtgtaaggtgtgttgttctgtgtaatcactatctgtaagaaggatttcttttgctaatttgtcatgcataaaaatacttgcaggttcagaatagggtgacctttccacttggcgaatatgcatcccacgtttttctactttcctatttatttttgagagcgattctttatgaaaatattcttgattccgtttgtctaatcgttctttattttgatggaaatactgttgtaagcgatcaattgattgttccatctttgtatctatttgttgttcttttgatgagcgaatagacgagctagtgcttggcacttcttgtggcaacggctccaaagataaatcagttgtttcttccacagctatttctggtggaacggtagtatccaaggaaagaaattcctctgcaggtttcgtgaacgcatcttctgatggctcaggtcgccagtccaagtcactttctctaaatccaccagctcccttctttttttgacgtagttctggatgattttttgcttcctgtaaaattagattccctattcttgaatagaggccattctttccataaagtttttgttcaaagtaggtaggttcatttcgaggattgccgtaagcttcttcgtattcgttggatattttttctagcttaggaagtatctttgccattaattcttgcccatcatattcaagaaaatgagtaatcagttggtctacttcttgtttaaaatggtgtttctccgcaaagccgtatttccagaagtattgattgtcaggcagtttatctagtaatgccaaaaacttttcttcataaataccttgagagaattgttccttacaagactctgccatttttttctgatggttaagacatgtttctagcatcgctaactgctctttattttgcattaattcattgacaaatactcgcttagtcgcacgaatatttttctgtaaaaatttccctttgaattgccaaccggatttactagggtctttcgggtgtgtgtaattgatccattctctggtcggatttttttctacatacccgacatggatatggatattgtccgtgttgtaatgaatggcacctgtccactcccctttgagaccttctttcttttctaattcctcgatcgctaaacgagtggcttgatacaattgttctttatttaggtgattggttttttcatctaaatagcgatggtccactaaccactcattgcgaaaactgaacaccatttgccacaatggagacttatttttttgcgcctcctcaaagtagtttttcatttcctgaaccacatgatttggtgctttatcatatgcttttgtaaaaagcgccgacgttttttctggattagacatataatcgttgtaggtcgcaaacattgtctcgttcccaccttcaatggcggagacactatccgactgattggttggagaaaatgcattaaaggaatcaaagtgttcgtttctggttgcttcatttctttccatataatcaaggtattcttgatacgtattggaacctggcataacaaaggcacttgttaaaatgataccagccgttttcttactcatcgtctacggaataattagaatattttttttgattcatggccgcaatcatgctcgcttctcgtttctttgccaggatttcttttgtttgtgtaagggcaaaagagtcctcgttatctcgcacagaaagttccattgtttttgccagggcattgaataaaatgttggttatttcgacatgttcttcaatcacagataataattttttattttgttttgtaagagacaatacttctctgtgcgttgaatctatttcattttcaacgatgtctaacatatactcaatgcattctcctaattgataatgtttttttgcggcgaaagtattcaatcgctctttcgtttcttccgtcatataaatattttttggcttctttttattcatcgatttttgctcctctctttgtcatttctaatgcaggtagaaagaactcacgcaccatcaattccattccttgatgcatggtttcaattgcttccattgtgaaagctttataacgtaattctgtctctaaatggaactcgtcataagcaatcaagcgcaacatttctctgagcatttcgtccctacctgaatagccttttttcttagctaccgttactaatcttttggcaatttctttatcaatatttctgatagttagtgtaattgtttcatccattttatattcactactccaatcgttttctactttattctaagatattcgcttaattgcgccttgtatttcggaagagcataagggggaatggggggcacacaaggtgccccgccttgcagtgcaaggcttcccggtgtattacacatttgactaccactagcataatactagcacccgctagcaggtttctagcactcatactagcacattactagcacccactagcagagttttagcaccgactagcacattgctagcactttcgctagcaggtttttagcaccagctagcacattactagcacccgctagcagaattttagcacccaaactagcacattactagcacccgctagcaggtttttagcaccggctagcacattgctagcatctatttttcttgtttcataaggaacctttttttcttttccgcaagtttttttagtttttctgccatcaatttttgttcattttttatctcttcactggctttgtcgtacttctcaatctctcgtttcaagcggtcaacttcagcttgtgtttcctctttttctttcccaactttgtattggatttcctcggaatattgataaattttgtcgtaaattttacttagctcttcttcaatttctttttgactagtggctaattttttctgtctacccttagtctctttttcttcttctgatatgacataaataagatagttctctttgggtttttccgttagtttttcatttgttttactctttcgaacatcccaataaagtgtggcttgctgtgaattatttttggctgtttcggcttgtttttcatccacttggttcacagacgtgggtgcttttttctccgcattgtacccaaaatcaatcgctaatagttgccatttttcaggaatgttcgttagctgaacaaggtaataattttcaattaatgggactaattttgcctttactgtttgttgttttgatacttcccctgcaaagacaacatattctttattgactaaatcttttccatcatccacatgtaaaaagatttcggcataccctgttttttcattcacttctcgtgagagaacagtgacttcactagagccaatttttgtgacatttgcttgccctatcccactgtccttaagtggactatcatcttcaaaaaagtttcgggagaaagcaaaaaaacagtacccaaccatcgtcaaaagccctataaaaagataaagttttgacgaataattttgccatctttttttccatttgttgctctttttctcccctgattgcacacgatctcgaaaattttcaatccgttcttttatagtgtttatcttctcgttcatgggcttcactccggcataaaataattatttggtaggtctctaggggcaacttgttccgtaaaatctttgattttccagtggttattcttgtctttttccaatttgaatcgatcaatgtatttcacatcaaacggagcaccattgccatgttttgtggtgacaaggatacaaccaatcatgaccgcttttcctgtgacgccatttagcttcacgtaatattgttcacttgctgtttcttggtcaattcgaaaatctgttttgtaatcattcacccatgcggggcgaagtttttttgataagttaggcgtgacaatctcttttaaagtagctaatttcttttctgctgtgtccgtatttatgtcataatagccagcacgaaattgttccccaatcgctttcaaattttcatattcttggtgagaataggaatgtttttcaatcggaatttctttagaaggctgccctactttttgctttttcagttcttccagttctttttctaattgggttgttttttcttgtgattgttggacttgttcagcctgttttggcaataatactttttgtgcatatgtgacggtaccacctacgcccaagactaacccacaacagcctgtcacaagatatttttgtatcattttcaacagtttttcctcctaaaattatttatttttccgaacaatgcttcggatttttgtaatgtcataggtacgattgtattttgcgacaaattcccctttttcgccattttgctcataagtagagaagtcttgtccgccattagaaacactacttataatgcccgtatggccataaatttgaggagttagaataccaccggcataccaatttactacgtcaccaggttgtaattcagacggtttcggctcgataatcacggtccaaccaaaggccgaccagttataatcatcccctattttttctgcaaattctttgccactatttttcaactttgggccccctaatttgtctacataataggccgttaaaaagtaacattggccattatcaatctgagtattaacgaccgcttctaatagttgaacatttcccccattgccttgatttataccttgttgcatcgtcgcaacatattggtaaatcaattccgcatagaacatatttccatataaaaagcgccagttccctcttgaattggcaatcggattggtgtagattgttttagctccgcctgcttgctgactagcaaattctgcgcctgcttcaaacgaatagggtcgatttttagcgtgcagccaccctaaaaacccgcctccgtaattgtaggcctgtaataccgccttatggtcttgaatgccatattgtttggctaaatctaaacaacttttataatgggtcaccccttgacgtatggattgttccgggtcatttattgtatttggtgctaaccctgcactttcactggattgaaacggatcgcccccacgtcccccggattccaccatgataatggccaataaataagggacttcatccggaatccccagttctttggccactcgttcaacgattggttttaacgccattacttcaggtgggagccctatattttcagcgggagataagttggttttctcttgcgtttcttctccaacaatagccaataacgttcgttgtgcttcttggacaatcgccagacaaacaagtccaatggagaacaccgttactagaaaaaggccaattttccatttccatgcgtttttcatactgatacctcttgttgtcgttgggtttgttgttctttcgtccacaacgcctgggcttttgtctgttctttttgttttacttgccgactaactaatttgcctgttttttgtttttccaagcattcattccagtctccttgttccattggcggtaaccgtaaagaaagatttgctgtttctttcaacgtttctgactggcaataggtttggtgtacttgctttacaaaatctcttccaggtaaatcgttattaaccgctaaaacaatttctccttcttctgtccctaatacagcagataaatcatggtaggtttgccaaagggtctcttcttttagaccagacaatgaaagaaaccatgtattggcaggtagattgtctttttctaactcatacaacgacaaagattcaatcggtgcttctgtcacaaacaacgtcataggcgagcgaaaatctacattttttccaaataaaaaaccacgatttccgtggctgttttctgcaattcctttaaagtattttcgtttcaattccatcgtgccatcggcagttgttttgattcttttggctaaaggaatcgcataagtaccttgaatatctgcacccacggggatccctagctgccctttggcaatttcagagaatttaaacagaatgttatggcggttgtctgaactaacgagttttttatcgacaaactcttgaatcgtttcttcggataaatgacgggattttaagtagtcccttccctgggcatcaaaggtacctgtatcgtaattgcccgccttagacagtttttctaacgtaaaaggcgttggcttttggataggtttagaaaaacgacgttcttgattagtggtcttggtgcgttgttgtgaaaactgatactctaacaactctgttacgacctgttcatacggttcttggtaaaagatcatcacaaattctatcgcattattataggaatttattccctgagaataccaattcaccacgcctgtttttacattggctcgtagactatcatgcagcgtatgttgcataaattttgacgacactttttcgaaagtctctcctcttgcttgtaaatactcgtacatattggtacgtctggcgacggctatttgtttctttgaaaaaacaggaatttttggcatttatctgcacctcccaacctatgaactgagaaacgataacagaagataaagaaaaaagaccgctactaccactaggtagagccgccttgttcgaacaccttcctttttttctgtgccaccaaagatcattcgtttccaattcctctgtatcttttgtcgtattgtttgttttttaactggtttgtcttgtttttccatctttacaagcctccatcaaagattttcttttctgtatcagataagccataacgaaacttgatattctttgcccctttaatgtttaacaaaatgtctcgttcttcaaagccaataatatctgcaatatcataggggcttaactgattcccaaaaactttgcgtaacaactcttccgacgattcatcttgtttgaataaaaaacgataggtggtgagtttaaagagattgaccacgatttgagaaatttcccccatcaccccattgttgtaatctgggaacgcatccgcaatatcatgaaagatataggtttgccctattagtagctttcgcccttcccgattgtagcggtcaagagcttttaataattctttgttttgtgtacgaatcggattatgaaactcgtctgaagtaatattggagtaaatcaactcgtccactcgtttctgcctacggtcaaagagatacttttcgcgttgtcccactcgaacagcttcactgaatgccgccgtatagagattataatattgcgcattgtacgtggatatatctgatttcactaagttttccatattgaacgtgaccagttttttgtcaaaaaaatcaaaagtagacttttgattaaaaatagtaccagattctgtgataaacgattctagcttatttatcaattcatacattgattgttttgcaaacgattctttgagtttgttgtattcttgtttcgcatagtctaaaatatcggaataaacagggtactgttctgccgcatattgggttattttactttcttctaagccgtgagaagccatatacgctcggtatccatcattaaacactcgcttggccgtcgtcattagtgggctatcaaaggcaatgttttcagctaaaccaaaaactaaccgcatttttaccagatttgtttttaacgactgggcttctttggtcttttttgtggcggcatctatatcggaacgatagatttgacaaggatttaagcgaacttctcctgcgtcaaaatattcgcctcctaaagcttccgttaaacgtttggtttcgtcactgacataaaatccatagtgaatattattgtattcgattgcttgttttaattgttttttggccgctgttgttttcccaaacccttgggcaccgataatgatactactataggatttccgcaagctatctttatgtgtggttgataaacaaactacgccagaaccgtacaggggaaagccactatatggcgcatctgaatcaatgtgattggaataattaaacgcatagcttcctgctagggctgttccttttatttctttgccttttcgtttaatcagtcgtccaccgtctttaaaactgataaacgaggctttaaattgtcgctcctgttcgtctaagaaacaagcagcttggaattgattttttcgtaattttcgatggacttcttgttctctttcgtctaatgcttcaatcgtaggctcacttaatacatatcggacatgaatttcttttaaaacgtctgtcgcttctaaaatattctctaccgtagaatccaatttttcatactctttgcgggctttttttcttgagatacggtcttttgatgaatagactcggtcttcgtattcccctaagcttttatttaagctttgttcgactaatgggttggttacatcgatggtatggacagatacagtagacaacacatgtttcatacaaaacacttgttcaccccaaaaatttgggttgttctttgggcgataaatggttaaattcaacgttcgaatatagccattgtttatttgtaactctctcgaagaatgcgggcgaatcccgcccatcggttgaatactgccgataaataacgggtcataaccttttttctccaccattttttgtgctttttctggtctgccttgttggtctgttccatgataaggaacccctgttggtaacggtgccagcggattgtagcgacggaataaaaacttgattttttgtgtgagtgtcatggtattaatgcgaaaatcagcactttgtgcttggcgaatttctcttcctacttctagtagttcttcttcatcggctgcaaacacttgtaaatagactgtatcaatcagtcgtgtgttatctaggttttctaaaacagctaaggtgtgccgttgctcttcccgtaccatcggacttaatgcacccattttaaaccgtcgggttgcatactcaatgttttcagacatatcaagcggaaaacttgtaaaaataaatgtaatatctgagtgaatggtctttagaaaggttagaaaatcatcgatcgcagcctgcctctgctgaaggcttccttctctggcggaagaatcttctattcggtaaaagttcgtcacgcctttttctagggcaatacagtcctctgaaataattcttcgttcagcgacaaatgacaagactgatttttcgacctttttaatcttgggtttctttttttcttccgtagtatccaccaatttcagtggttcttctaagagttcatcggtattgatcacttctttttcacttccttatacaacaaaaacccatcagcgtcgttcttctactgatgggtttcctttttattattattcaatttgtgccatttttttcgccacttccaacgaagataatcgacgatttgtctgcgctgtgtggcttttttataatcgtgttgcaaaaaacgtaaggtttcaaaaaaatgagccattcctggttgttgccaattttctttcgttagaaattggccacgagtacgctttctttgttgccctggtcgacgatacacattcagaatataggcaatggtcatagggggctcactttttttgcgataaggtttggtagggacattaattaagccacccttcagtaatgccttccaattatccggatgttcattaatatacaaccgcattggctcttgcaagtcttttggcaactgcaggcgctccttttccccatccaaacgttccacatgaacatagacaaacaatggtgtttcttcttgtgattccataggaacactcaaaatggtaggtcgtcgtctgaaatttcaatcggactgtttccttgctcaaacgggtccaatggatcaggtttatctgttggttgcttgtcaaaggttgcttgtcctgcacctgtagattgtcctctgcgctgttcgtttacttcttttgattctaacaattgaaagttttctatgactacttccgtcacatagacccgttggccttgttggttttcatagttccgtgtttgaatccgtcctgtaagaccaatgagtgtgccttttctggcataattggcaagagattccgctgcttttcgccaaataacacaattgataaagtcggcttcacggtcaccattttgattggtaaagtttcgattgacagccaatataaactgtccgactgccgtgccactcttggtatatcgcaaatcaacatctttggttaatcgtccgactaaagtcaaattattaatcattttttcttcccttccctcattgtccttttcttcgctcgttcagcaatcggttggtcttgtaccctaagacctatttctagttcacccattcttttttgtacactatctctataattttctgttcgatttattatttttttcatggtttgtccctcgttcattttttttaggaaggtggtgatagtctaaccaatacgacagggtacacaaaagaaacgccccccatccaaaaagagttagtttcctttcatcatctccgggggtgttaatccactcaatacaaaaaaatagccccatgtataagaatcctaagataccaattatccttcccactttttttaatcgcttcgcatttttttcggtaataacagaaaagaagcataaactacgttggagtaacaataaaaaagtggctaaaaaaatcaagaatagcatccattctacagcaaatagcttccatcgatgttcaaaaccagcaacaaacatagtaaacactaaaaaaccaaggcaaaggccagcaaataaagtcaaaagaacagtcagacacttttcaataaattggaacagtcgattatctatggtacattcactcctttagtaagcaagagtatcattatttggtttctttttcttgctcttcctgcctttttacttccttaattgaagagcgaattagcattggtatagcgactatagctaataaaatcccggtccaccaaataatcgaatgcattcgcatttgtcgaccaacatttaatagttgcataaacagaagaattgcaatccaaaaatttaattgtttccccattttcttgagcatacgcctatttatcctctccatttaccgtttgccagtacttaatttggtctggcttaaatcctgaccaatattctaattcctcttctgtttcatcatcaatgatttttattagtggtaggctttgtataccatattttgcttttattttttctacttttttctcgctccatgtccgtttctgttcattgatactattgacttcaattgaatttgtttcctctgaattcccataatacgtattttcatagggcaagcctacttcgtccattactttggtgctcattttacactgcacacagtggggttttgtatataaaactgcatgtactttattaaccatcttctaattcctcaactatcttatttttagtttgtttgttgttattatatcaaaccaagagagagtttcacattatttcatccgtcattgcttggtcttcttcggctaattccgattctgttgccatcaccatcgacaattcttcttcatcactaaaagacacttgggcaattgggtgatacgtttgccgattgttggttaatacaatccataaccgctgataatttcgcaaccgatagttgccaatactgggtgctaaccaaaaaagcccaaataaaatgacaaacaaaaaagcatatgtccctaatgggccatacgttttttcctgtaacccagtagccatttgaaacaaaataaatccacagacagcgtcttttgttaagattttcccataaaactttgcttgtgtaaaaatttcttcctgtatttcatgcatacgttctacctatgcttagcctttcttatttttttgtcgtttatcttttggtacttgttgctgtttttgcttttttcgttgttttagccactcgttcacgtcttggccaaattctttgtttcgtttgtatcggtctacttgattgccaattggatttttttgattcttctggtgtttattggtgtttatcatgttgtttagtttcttcttgaacggattttccactgattctgtcggagattgctccgttggtgaagcttgttctccacttgatacatggtgttcttcttgctgttccgcttgactttgctgttcaactgcctctgtatttttaccagtagctaacgattctggttcttggttctctccagctgtgtggttgttatctttcggctgctctagttggctagtctcttcatctgcttgatttttctctgtttctgtcggcaagtctatagtatgttgctctttctttgttccatccccttcaacgctagattctgtgctctcagaagcatcgttttgatttttctcttgacttatttgcggatcgttgggctcttctaaatcttttccaccagtaatggtcgtttcttctggtacttcctgattttgctccttttgttgcttatctggcttgttatgttcggtttcttttccttcgtttccttgtaattcattattcagttcttccgcattcgttgggtcattgtcccggttgtttagctgatttaagttggcgttttcatcgtttttcgtatcggaccctcgtaaaccatccgcaaatcctgctaaagcaactgttccactagttcccgcaccagctgctgttttcacaacactactcattttatcaatcgctgtttttgcacccatgcccattacaaatgagcctgccgttgataaaccggcatcaatacctagtgtcttttgaataatggatggcccatcgtaaataaaccaggcgccaccgattaccgcaaagagtttggctaacatggaagattgttgtgcaaaaacaaacgcattgtatttaataaatacgtagtacatggaataaatagatagaatcattacgaaccctccaacaatctccattaagaccgtcttcgctcgtttcgtatctcgaaagctaaaaaaaatcacaagatttgcccaaagattattaaacgcaagttcaatacccaaccggccaactcgaacaagagaaataagcatggagagggctaaaaccgatagagtgataatcaatggcaaccaattcactcgccagcgataatatttaggggcaaacgtggacttgattaaccacccaagaacaccgcccccgccttcatcaagctcctcaacctctttcccttcttcgcttttcttattgactagtttatatttgaggacttccccatttttgacatcgtcagggtcagtaatccgttcattaatatcaaagcctttcctgtctgttagattgttttttatttttggatctgtggttttccactcgccatccgctagcaaataaatatccgttaagttttctttgaatgttgaaaacccaatgctttcttgtttggtatccaaatctccaaccgtcgcattgatgattttcaacccatctcgcatgatattgggtaacattaaggacattaggagtaataacaagacattcattggaatgtctcttgtctgattcgattttcctaatatcaataccaatccgacagcaagtattgctagacctacgccaaaggctttaaaactgattaatgtgtctagcagactgccttttccttgcatagaattgtcattgtaaaagcctaaaaagtccaacattgcactcatcacacccgttaagccatcgacaatccatagcaagaaagaaaccagaaggtctagtaccctccgacctgcatctcgcataaaatcagcgatgtgtaaataatccgagaacatctctaaaatcttaagaatttcttccgtcttcatccagtcgcctccagtccttcagttgttggatcaccacatttactgcactttcgctgaaatttgataaaagacagctaaaatacgaaagcaatgtgcctgcttctgcgattttttcgagttctgaaaacgtctgtgtgtccttttttccaaccatttttatgtttgaaaacaacacttgccgttgcttttctgtcaagatttcctttaccggtcgttctaactgcttgtgatacagctgttctaatatctttgcttgtttttgatattttttcgttgaaagttgtgtttgttcttctttcaatgctgctacttcttcaggcgtggccactttggtttcttgaacccgtaccgctggttttttgtaattaggaatcggtggcacaaactctttcggtcgctgttgactactgtctggttctaatagccaattcaattcctctaattctacttccataaattgattattcacagggacttcttcccatgagactttttccattttccgatactcataaaaaggaatcaagtgggtatcattttcatacgtattaagaatagggtattgataaatcggatttccttctaagtcccggtgtttattaattctcaaaatgaccgattccccttcacgtaagcgttccaattcgtacgatgccaataaatcaatccgttcagaactctctgtttccgttgacttcacagacaagggatctttgtggcgtgtttttgagtaattggaccgttcacctaatcgtccagcgatatatttattggttttatccgagcctgtccgaatataggcaagattccccgtactccctagaataatgtctttggtatcttcatcatataacgacgaaagctgttgaatatcttgtaagactaagtgtgaaaacaagtgacgacttaaccccgcggtccatttacgagctaaatcgttgatggctacgcctagatttccaccttcttcataaataaaatgcacatctcggtaacattgtgattcatcttctaagttacaacgattgatcaacacctggtaaatctgttccaaatacatcacacctagctgattgtttgaggtatccgcatcacttaaaacaataaacacagctgtaggctgctctctgtcaaagccgattttttccatatcaaagccatcatcaatggccgtcattttagcgttcaatgacataagaaaaggttgcaagtccccgtcaaagtgggtaatgatgtttcctaaggtgacatgtgcaggcgctgaggccataatcgcatcataaaaacgtttcgcagggtgtgttcttggcaattccccgaaaaagacgtccaattcactctttccatcatattccgctaataaccgttgcacttcgtcaggctcttctacatagcgtttcaaaaattcgtgtgagccttctttgattcgtcgtttctgcatttcattcactaccgtataaatcgtgtacggattgactttgctggtttcttcttcctcatattcttggtcagctaatgccatacccacactcacaaatagattccgacaggcttttgtccagaatccaccgtctttcccttcgttcacttcccgaaaatacgaatgcgcacactgcgtaataattttttccgcattggctaactgtttttctgcttgaatactgcaatttaacgcttcacttttcttcccagccacttttaagtcggcactttcttgttttaagcgtttgtaatgacgataatagttgttgaacacgcctagtaccggaattgggtcggaatagtattggttgacagtattgacgacacgtatatgatacccacgacgttttagggttttataccacttccgtggctcgtcgcctttggttgcggtcatgacaaaagacgcacgatttttcattaatcgagctctcgttagaatatcaataaacgggtccacaaagtagattcctttcccttgtcgggttccggctaaagtaatcgtatttgaatcagttgtatctacataataagaaaatataccagcttctttttctgcagctgtttgtggtttcttgccgattgggtagcctggttttccatcaaaataatcttctgtttctgtaaaagagtgaacagctgccaaggtgtactgtttgtctaattcagttgttttttcaaaatccatcgtcccttgtacatgttcttcttccaatgaacgaaacgaagtatataggcgataagcaagaacactgaccgaaacaaaacaagccaaagctaagagaaaataaacaaatggaaattgccccaacgggtaaaaaaataaggtgtctttaaaagacacccattgtacatcaaatagtgagccgctcgttaacgatagaaaattttggattacccaattgccaagcatgaattctatcaagaaggtcaaactcatgcttgggagtaaaaatcgttgatctgctaaaaaacgaagactattttgtttggctttttcataatttttctttttggttttactactttcttttttgcgcaacatcattccaccactctttccatggcttttctttgaaaaattgtcgaacataaggaatctccactaaaagacaaagaatggccggcattagtggaactgtgtatcgtagattttcttctaagaatgaggagtaggtaaaaacaagcacggtgaacacactaaaaatcaaaaagaaaaagtggacaaccattgacattgcttctttatgaaatagcatacacccgcacgtccccactaaataaaccaataaaaaggcactcaaaaaactattcactcccagccactcctttcatgttcgttactggtatttcgtagtctatccttctcggaacaatctcttctaagtgaatggataaagtaaatggcgtatagcggaaacggaacaaaagttgcactgacgggattgtatacgctgtgtgccactttcctttcactaactcttccgtcgttttacggcaacgtttgttttcttcacccgctaaaacaacatagggttgccaatctccatggattagccattcgttggctgtatacgctgttttagatggatataacggaaatatcccctgtttcaattgttcgtctttaatcgaattaaatcggcgaatcaacaagtattgaaccagcatgatcaccaatagcgagaaatcctcgctattggcggtctcgctaatcccaattcctacgagtaaagcaatcaagcctaacgaaccataatatcgactgattcgttgaacaattcttttaaccgttgcccactcatcttgtgtttttaggacatagtccattactgcctgtaggataaaaacgaggaataaaattggcaccaagttgtcatacgttgccccaaaaggactcacttcagacaatcgtccctggccattttttgtggcgacatagactgtgttcccaagtaactgccatcctttggtggctacataaaaaacactcaacgcccatatgccccacgaaaggaatcccatgattttgcgtaggatcaagaagcagtattctattcgtatcctttttttcattctttttcgcaccacccttctaaggttgccttttctctaggtgaattttcacctaacccctgttcaacctttggattacggccgataccaaaaaggaatatattcttattttcttttgaccctatataaaaaggattcgggttcaaatctaccttttgaaaattatgtttacttttcttgattggtaataggtgtctccaccattttattcgttggttcatctattttcacttccgtttcttctttttgtgcagttgtacctatcgttgaatcagagactgtctctggttcttttggttggtctttgattggttgtggtaagtgagtaaagtctttttgtacgtctgcaacggcttgattttgcgtagttgcgatttccttcacttcttttgcggtatcttgtacctcacttaatgtttcttgtgtttcttggctctttgcgacaaccaattgttgtgcaattttttcttgattgttttgtacagcaacagcggctgcttctgcttgtgcaacttctgtttgaacattgacagccacttctgtattggtttgcacttcatcaattgctgtaccaaccgtttcttttgcctgttctgcttgaggttgcactgtttcttcgtagttattttctaggttttccaagttttcatgcgtttttgttgcattagaaactttgttttcaaaatcatttgttgcctggttcgctttttcttgggcgttgtgaacttcgacaactttttcttgtagttgttggtatgtttggttatacaaagttgcattaatctcttctacctcattgttctcacttactaaggttttaatttgttcagataactgattatattcatcgactaaatgcactacttctgaccaataatttgttgtttcttccccattcttacttaattcttccacttgagtaagttgcgctaactttttctgcacgttttctagttgatgattaatgttttgtgctttttgtgtggccgctactagttgaccttgtgattttttaatcaattctgaaaccgttggttttgttggttgttcgggttcaactggttgatctggttttgatggttgctctggaacttctggtattaccggtaaatttggctcattaggtactagcggtttatccggaatcactggtttttctggtaaaagtattttatcggttgtatctgttttccctggtaatttttccattggttcacttggcgttttctcattagctaacgcaagaattgtctcccgctgtttttcttttttgttcgtttctcgaatcgcttccttacggtcctgttgaacaagcgcattcgctagttgtcctaatagatcgctttttatttctggtatttccacaccaaagagttttggtttttcttcttttgtacgttcaaaaccgctaactacttcagctaacgaatctttcgtttgttgagactgcttactttttttgtctttatccttgtttttttcttcattttccgtcactttccgttcccaaggggactgtttactttttgacgtttgacgttcttctttaggttttggaccttgttgctctgtctgtgcgtccttcttttcgccctggttgaatgcagcataagtcagcccgcttcctagtaatgcgacagaacataacccaattactaaatatttttggtgttttttagcggtttctttttgatttccgttcatttctttcattcctctcaattgttgtgtacaaaaaaggagctattctttttagaacagccctttttttgcttttttatttactttctcgttcgttatacgtataatagaatatgaaaagaggacatgctcgaaacatgtccccttagagtaaatgaccgatagaagatcggcagcatatattttgacgatacaaaaaaagaccgccgtaaacccgctaaagtctaccgacggtcttttttgttgtcgtcttttttgcctaatttatagacttgtattaatagtgtaagtaaggccaacacttctaatacagacacaactgcacaactcctttgccagtttttctgatttactatgagtactctcataggcaccagctcctttgcggtggatttatgctgccgtcttcaacttccatttactctctgtgatcataccatatttttactcttttttatataatctgtaaaagtagtcagtcgtttgttgttccaaatgctctagttgatcttttacttctgttagctttcgattaatgtctctatactctttttgtagatctttatggtctctttgtaggtctctataattttggtgcccaaacacaataagtatgagcgtaaaaagagttatgagtatcaacataaaaatacccagttgtaacccattaattgtcgtaagtttattcataatttgatttttccctccgaattaatgagcagactttccaatttgttccaagtttttcagccatagctggtaattatcggcagcttcttttcgctctttttccgataactctttattttccttatctttggcgtatttttctaacaagttatgaatacttttggctactttaattgcttcgtctaattcattatccttcagtctttcgtttattctctccgcttcaggtatttttcgctctctaagaagtttataggcctgttcgatttctttacttttgatttgttttgttaacgtaacgttttgaatttctttattaataagctttgcttcttctatcttaccttgttctaaaaaagcatagcctaccattgcctgaacgtcactctcctgtggtaacttggaaagttctgttgctttctgccaatctttctctaaaaacgcaagatatagctgagctaactgtgtattagaatgttcagctattattttcaaaccagctttatcttctttttgaaacaactcctcaattagctctggttctttctcaggatatttttttactatttcagcgtacttttctttattgactaactgctgatacgtaggctctgaactagttttggccgtcgattgacttcccgccataaatttccaaccaatcacaattaagagtattcctatagcaaatactcccaaaattttcagttgcttttgagaaagttttattggaaagactacttgctttttccttttaggattccccactttttttgccttttttatttttttctcttttttgaaaaagcctatttccttctctttgccagatcgagccttggcttcctgtggattcttgaaagagagtttatagaacaaattttcggcttgttctgcggtcattttcttttgtttgattagttgattcagctttttttgtatgtctctttccaacgtccatccttcagaaagtttagtaaaggtgcctcgataaaagggatctccattgacttctaatagttgaaaagttactgtctcatcgatttccatgtattgggtaatctcaagaaaatctaaaaatggaagtaattccaacgatggttgtttagcgagaacctcgacgttggaagaaaggatttccacttcgacagccattttttatcctccaatccaaccccatactgtgtctttgatccatgtgaagttaacgattattgcggcaccaataaaggctccaaagacccatttctttgcccactgtgctacatccattcccaagaagcgtgcgccgccataaatcaataccgcaattcctagtgcaggattggcaaactttcgtagttgatcgccaaatccttcttctacacctcttaccgtactttctacatctgctagtactggcatactcgtatagacttcaattagtcctaatgcgacaatcaattgaaagactccaagtgcgtattttactttcttttctacaaaatttttcataaatagttttcctccaaacagttttttattgattgtgattcccttgtttttttcgttccaattctttggctaataaacggtcaatgatctctgatttttctaaaagatagttctggtgttgctcatttagccattcttcataggaagtaccatttaacttcattaaagcttgtaccctttttttggttgtgctatcaattttagttgccatacttgttcctcctaaataattatttgtcgttcttttggcgctacaagttcaaacggaatttctaattgtgctaagcgttcacgctctcttggaaaatatcttacggctacttttttgatatatttcttcttaaatccatagttttcgtaaatataaccaaaagaatcaattgtttcgttataacgctccactggtttaacggctatataataatcaaaataaaacaagcacgtgataggcgtttccacactgacctcaatttcactacttagcgtccataatagcgctttttctgtttcagcaccttcttgtgtcttatggcttttcacccatgcctgtcggctttttaaccattgataaccacgtttgcgtaacgctgctttgatagaaaaaccattctcaacaacggtacaataaagcgttccttgtgattcttctacccagctgtccaagtcaccgtatagagcgatttcttcttctaagaaacctgtattcaccatgatttcttgctctttgggactcacttttccttgttttattagttctgttaacaattcttttactattttttccttggcttcttcttcctcaaattgttcacgagtcacaacaatcacatgtgtagctaataaacgaaggagtgtcaataaaatctccgctggttcccgcaaaagattgctaacttctattacccgctctacttctaaataattcccaatggttcgcttgcgctcttttggaagtatacggatataaaaatgcttatacgcttctgcgttgagatacgtctgatccaacagctgacacaaccacttttttatgtcttgttcccgtacattcattaagcatcaccgtctttctctcctttggcgttcttcttcgaacaattcttcaatgattgttgcaccctctttggtcgaatttttgctcacttctgtaaaacgcattaaaaacgccatggcctcatcatgtgttgctttgggaaaccgataaaaatactctcgttgtaaatacgcccaaaattcgtcactgctcacactttttgacatatccttcactcccctgcctgtttttctgttcgtttcgcagttctttctctgataaaaaataatcatgataggcttctcgcttaattcgtgtttcaatgtaaaacattgggacttcaaaagtagagttttgttcgaatccaaacttgcttctttcggtatccactttcagcgttaatgtttttccgttctttagtaagtggataacatcgatctcatgaatattttcaggtgttacttggttatttgttaataattcaaaggtttttccttttttaaccttaatcatcaataggcgaccacgaaatccttgccaacgagtattgacttctttttcctgaatagctaactctttcattgcgacacttcctgttcgttcttttattttttccatcattgtcctttccaacaaaaaaagagaagcacgcatttggcttctctttacctgtcttcattccttcattatttttctgtttcttttcgtttcaatccaaaccatgccagtcctgcaagcattcctgcccctagtacagaaagtaacgtattttctttctcgccagtatgcggcaattctggcaccacacttgccttttctaccactaatggctctactggtgcttgcggtgtttttggtgttggtggtacaatcactgttttttctggtggcgtttgtggtttttctggcgtatgtgtcactaccgtattcgttttaatcttctcattgttgaaagattcttcgattgtgttgtaaacgtctcctgccgcaattcgttctacaccaatgaacgctttccatgagtgtgcaacgtttttgttttcttttagattcatcgcatctaaaaaggcttgactggccgtgattttcactacccctttgtcaaaggtcatcgtgaatagtttcgaaatgtcatcccctttattcactttggttccgtctgctaagacaaaattagaattggcaaacacagaccattggccactaaatttgtcatgtttgacgtctagtttgtcactaagcgaccattcttccacaacaccagcgtattctgcaggaatgtcactacttgtaaattcatagaagaatttctcccctaatttgattgtagcgccattttgactttgtttgtcaccgactttaataaccacgtcttttttagggttcacttttggaatatggttgacaacggtattcgttttaattcgttgaccaaatgtattttgttccgctgaattataaacatccccagaaacatcagctttgacttttgtagggagtgttacacgcaattcttgcccaccatgcgctagaataaaggcttgtgggtctttggcagagattgtcaccgtgcctttggcatcgtcccaagagatcgtgaactggttggtaatgtctacccctttagaatctttgacacgaagtaagtctttgattggtgtcactttcgtttcgtcgtaatcatcgaagaaagaaacgcctgtcgcaagatcgactgtgtcaaaagcaaagtctttatcgtacccttttaagtcccaggtcatttcataagaaagaacatcaccacgagccacttttccatgattaatgtcttcccctttcttgttatgaacggctttggttggttttggatcatcaggtgtatgcgtcaccaccgtattagaacgaacaagttctttgttgtagttttctgtttgcgtattttctacgtcacctgttttgatccgttcgacttccagatacacagaccaagcttgtttgcctactttattgcttccttcatttaacgctgccaataatgcttgattcattgtaaacgtcaagtctttattgtctttgttttctaaaagaatgtaggcagaaatatctgttcctgcttttaacgttttatcccctactttaaggtcatagttcgtaatagcgtgccattttcctgtgaaacgatcatgggtcgtgtccaagacatcattcatgccccattcttctgtgattccgccatagttggctggacgttcggaagatttcacttcataataaatttttgtttgtaacggaatatctttatcatgtagagaaacactgccaactgtaccgtttttatctgcttttacatctttggaaggattactacctggcacatggttaatcactgtatttgttaccgtttcaccatcgtttgtcagctgaacagctgtattttcaaaatcgccttctacatttttcactacaaacggcaagacaagtaaatatttataccccattgctaaaacaacggagccgtctgcgttggttttcatcattgctgtgacggtgttttggtctaaattaagatcataagaagcggtcacgtctttggcttttcctgaattaatcgctgcagcaacagcttttaagtctttctcgtttagacttgcgtctgcttgataaactttcactttggataaatcaatcgtcactttttctgcatcaaaggtatctcgaatcccttgttttgttaccgtttttggatctactttagcaagttctgtcgtatcccctgtcacaatgtattgtaaagaatcgccacgcttcacatttaaatcattgatatttttctgaccatcagtgacttctttattcggaacaagaacaggaaccacattggctttgtatcgattgaattcaattgttgctttttctggttcttttggattccctttcttttggtatggtctaattgatttcgcatttaaattggtactaaaggcaaaccattgcgcaccagataggttgacttttcctttggttgtcatcccgaaagagaaagaaatacgtccaccctctctagctagaccaacaccagaaccatagtacgcatttttatgacctacagcatcccaatcactattttttagtcctgaaggacctgttccataatcaaggtcttcggttgagtagaattttccatctgcttgtttctttacgtaggaaccattaatatacttgaaggcattttttgaaccaaagtctgaaacaaattccgcatgttctacactataatttgttcctagactagagtttaatgacgataacgcataggcaaaggcatggtctttctctggtaaaacttctttgccattagcatcatataatttaatggttaagcgaacttttacgtccttcccattggcatttttagtaccaacaaatgcagtaataataggatcgtttgaaaatactgcatttaaggtgccgctttgacttggtgcagattgaagttcataaatgaattctgtttttgtgatttttcggtttaaataactagcatttaagcctgtatacgtgacattggccggtttgtttttttctaaaagaaccgcgtagccgcctttaggaccaaactcaacagcagccacttttgagctttggaagttgcctgttgcttttccattcatatctttacttaattttgtaaaaatatctttagattgtccttggtttactttgttaaattcggaggctttaataaacttgccacctgtaatcttgtctattttagtatccttagtcacaatacttgaatcaaaaactaagtctttgctgattgcttcattaacatagcctttgtcattcttatgtttgttgtattccgccacttctttttcataacgctctttttccgctttgttttttgccgcaatttctgcattttctttggcaattttttcatttttggcttttaattcagctgcttgttgggcaatctttttcgcttgttctttttgtagttggtctacttctttttctttttcgactaaatctttagaagaaacgttgcctaaatcttcagttggtttttcaacgacggtaatgtttggatcttttttcgcctcatcaactgctttgtcaacgtctggtgtttcaaattctttaggaatagtcgttgatttattcgcttcattttcagctggtgcaacttctgttggctgccctagaggttcattggttgtttcagggcttactactggttgttcttgtgctgatttttcagctcctactgttggttgttggacgtttgtggtatcatttggggtagctgaactttgttcagcagcaattcctttcggcactacttcttctgctgtggttggttgagaagtagtgtctttttgtactgccgattcttctgatactgccgttttaggtgtttcctttcctgactgcaggtcgggattatcgggttgcaccgtcgttgttcctggttgcgtatctaattccgcggcttgtacattatctgtagctaatcctacagctcctaatacacctaaaaaaagaataggggctacaatccagtgtttctttgccttatacattttgaagcgtttctttacttctgtctgttgattcatgtatcattctcctcgattttttattttttgtttatagaaatagttcacgcaacacaaggggctcgttgctttttcatcattatttacattcctcctcacaaaaagagaaccgaaagtttttcgattcccttagcttttttttgcgttaaaaacatttaacgtgctatcataattgtgtaaaaagtacaaatcacttctttacaaatcttattcgtttagtcagtcggcggaaaacggctgacttttttgttgcctaaaattgcatagtcaggtactatttaagtgtctccatccgagacaatccatttattttttgttgaccagcggaaactggttggctcctaaatttggtagattcttctgcctttaatacgatcagccaaccattttggttggctattttttatttttcaatttattccaatgattaaaataaaaaggagcgacatatttcgctcctttgactttattatttaattttaaagatattttttactttcttctcgtttctactaataaaacttataatacccgcagctccaaacaaagcaaatatcagaccagctatagctaaccatttattatttttttctcctgtatgtggtaaagagtctggagcttttgctacctgtttcgtcttacgagattctgaatgtgttaatgcttgtgcttttggatgttctttttgtttacgccgattgtaaaattaagctagacaaataaaaaagtcatttgtgctacactcaagatagttcccgcaaaagaattataaggagtgaagacaaatgacctatacccatcttacatcaaatgaacttgcaatgatagaggcgtattataataatcatcaatctgtagccaaaaccgcagtactattgaatagatctagacaaacgattcataaagtttaccaatttttcaaaacagggcacaatgctctagattatttcaatcaatacaagaagaataaaactcgctgtggcagacgtcctattgtcttatcagatgaacaaacagaatatattcaaaagagggttgttcaaggttggacacctgatgtgattgttggccgtgcagagttttctatttcttgttctatgcgtacactttatcgtatgtttaaacaaggcgtatttgaagtgactcacctacctatgaaaggaaaacgtaaagccaacggacacaaagaaactcggggaaaacaatcttttcgtcgatcacttcgtgacagaggaaatgattattctaaattcaatcaagaatttggccaccttgaaggggatactattgtaggtaaaaagcacaaaagtgctgttattaccctcgttgagcgattatctaaagtaatcatcactcttcagccagaaggcagacgagctatagatattgaaaatcgtttgaaccaatggatgcaatctgtacctaagcatctattcaaatcaatgacttttgattgtggaaaggaattttcaaattggaaatcaatcagtaatatcaatgatattgatatctattttgcagatcctggtacaccatcacaaagaggtttaaatgaaaactctaatggtttattacgtaaagatggtttaccaaagcaaatggacttcaacgaagttgatgaatcttttatccaatctattgcatcgaaaagaaataatatccctcgaaaatcattaaactataaaacaccaatagaagtattcttgagtcacatatgcaaagaggaattgtctaacttaatttgacaattaatattagaaaaagataactgttggagaccaggtattttgtctgctgaagtagcaattgctactaacatttgttgttgctttgcttctcgttcaagacgttgttgttcttttgctacttgctcttgtaacgcttcttgtcggcgctgttcggattgttgtgcttctaagtctcttaatacaccttggtactgctgtagctctaacttcgcattagaaaggtcttcttgtgcttgtgcataagcaagtgtagcaacggcttgttgttctttaagttcttccaatgattttagagaaatagtgtatgcttcttctgcatgaactaatgttttttttgctttttctaaggctttaaccgttttttcataatttggttgtgcattttctaatcgagataacgcttgttcactgacttttaattgggcttgttttttgccgagtgtttctttggcgatagctaagacttcttgcaagctcttcaatgcttcttcttccgcacgttgtgcttcttgtttttctttcagcactttagcagtcgtttgttcaatcgcttgtgcgtctgcaacttttgttttcgctttttctaaaacagcagctcgattctgaattaactcattgattgttgccaattgatcttttgtttgttgcaggcttttttctgcagctgctgtttgacggactttttcttcgtggttcgctttacttttagctacaactgcttgtaacttagtcaatttggcgttattcactgacaattctttttcagcagtagcttgattggctttagtagtatttaagtcttgtaaactactatttcgtgcattttgagctttctgttcagcatttttcgcatttgttaggttgctttcatttgttgcgatttctttttgtacttgttcttttgatttaaagactggtatttttccttcttcaaatgttgattcatcaagtaaacgttctttgttgtatccaataatatgaattttacttgaaatatcatttaagtctcctgaaactgaaacagcagtattagtgtcctctgcacccaacaatgaatctaggtgtccataacctgagctctgatcgtcaaaaagcatatcaacaattgttttacgcgcagctttttcaaaatctagcatagatatttttccgtctacagtttcataatacccaattgtcagattttcgtatcggttttctcctggatatcccttaaatccattctctttcgctgctttattaattgcattaacatcatgtccatattctttaggattatcgtatttagcaacatcccaagcaaatttcatggcttgattagaaatcttcaacttttgtaatccgaatttttcacgaacgtcgttgataagtcctacaacataatcactcatttgatgcttatgtttttctgtaggatttttgacattgatcatttccgttgcttttgccgcatctgcttgattttcagggaaaactttatttaatgctaatgcttctttttccattgcttgcttttcttgttcagttaattttttgtaataatcaggtgtgaaattggcagacaagttaatccctttatgtccttttagctcttcttttgagctatctaaagtattctgcgcttgctttgttgctgtttgcttgtctttcaaagcattttctttcgcagttaactctgcctgtttcgcagctgtatctgcttttgcgtctgctactttttcttgactagttgtcacaacagtttgttggtctgcaactgcttgatcgtccttcgtcttttgatctttggctttggcttcttctttctgtttgttagccaattctgcttcttttgctgcttgttctttttctgcctttactttttccgcttccgcatttttcgctaattcttcaagcttgacttgttcttgttttgcagctgttactgcttgttgatctttatcattttgcactttagcagcagtcgtttcttttgctttttcatcaacaacagcttgttgttggttaacgtctgtttgagcttgctctactactttttgttggtcatcaacagcctgtgtatcagtagccacttgctctttggctttttcaatggctgaaggtgttgcttcatccacgacttttttagcttcgtctacaactgcttgttggtcagtcactgcttgttgactttgatccaatgcgtctttgttttgatcgaccactgcttgttggtctttaacagattgatcaatggtgtctttttcttttttcgcagtgtcagcaacttgttgtttttgatcgacaattgcttgtttctctattacttgttgctgtttttcagtaatggcttgctccgttgtttgtgtagctttcactgttggttgttctgaagaagcattttcaggtgtttttggttgcgtttgttctgctgcctgtacctcatttcccccaatacctgctacccctgttgcgactaagatacttaaccctgtacttgcgatctttttcattttattttcctcacttccgattttttttgttgtaaatgggatacccattatcttcacgccactgttttaatactttttctgttacatgaaatcgttgagcaatttgtttgaattgcaagccacttctctgatagctctcaaaagcttctttagtaatttgtttgtaatactgtcttacatccgcagtttctattttttctgcgagctcctgaacacgttgaaaacgctcggtgtgttcttttctatgccaatcagggtcttcattcattaatcgtaacatttctttacgccatattttctgttctctttttgtcatgctctcacccctcgtaaattatcatagcaaaagataactaccctgaaaaataataccctgttatttcgtgaaatatgtctcataaggaaacacctattgtttactggtttcaaaaaatcaagtcttttcacagggtttctagcaaccgttaccctaaactctaggtgagtcggatattgctcgctaccaataattggtaggtcgtggcaatctcaccatgtaccgtagcacaccaacttcacaatcattgtgtgggtctccgttcatactggagcttttagcttttctcctagcgtttaacgacaccctgatggcttctgtacccttgccccttcatagctacgctgataagcaaggcagcggacttctcgctgactattcagttgtaaaaaagaaagagttcttcttctcgttatcagaagatagaatgtttcttttttgtttggcaactttgctggaaaccagcaaacaataggtgtttcctgaatactttttttacacttcttcttcgtttaaataattccaaatagtagtgagtaactgatcaaatcgttcgacaatgaatacgtcaacatcattttctagtaaccaatccactgttatctcccaactcgcacctttttgcgcagctcgatacagatggccttggaagtcttgcggaatgactagttttttcttgtccgagcaggcaacaacaagagctgtaaaagttgtttcatccattccacaattttgttcataggaaaatactcgtatcacgtctccgtgatttagttcttctgcatgggtaattcgtttcttttccatagagtcctccttgttctatttactcagttacacttcctgtggtatactattcttaacattttattcattaattttttctttcaatgatgcttgtcagctagcggaaactagttgacttctttttttattcactttttttacaggaacaagggttaacttggtggaccctttttttcgttcaatgattttatttccatctttgtcataacaagaaatga